European Patent Application EP 4 268 852 A2, published November 1, 2023. Title: Variant adeno-associated viruses and methods of using. Applicant: Howard Hughes Medical Institute. The sequence listing filed with the application follows.

SEQUENCE LISTING (108 sequences)

SEQ ID NO: 1-2 - skipped (2 entries)

SEQ ID NO: 3 - DNA, 2238 bp, synthetic construct
  misc_feature 1..2238: note = synthetically generated sequence
  source 1..2238: mol_type = other DNA
atggctgccgatggttatcttccagattggctcgaggacactctctctgaaggaataagacagtggtggaagctcaaacctggcccaccaccaccaaagcccgcagagcggcataaggacgacagcaggggtcttgtgcttcctgggtacaagtacctcggacccttcaacggactcgacaagggagagccggtcaacgaggcagacgccgcggccctcgagcacgacaaagcctacgaccggcagctcgacagcggagacaacccgtacctcaagtacaaccacgccgacgcggagtttcaggagcgccttaaagaagatacgtcttttgggggcaacctcggacgagcagtcttccaggcgaaaaagagggttcttgaacctctgggcctggttgaggaacctgttaagacggctccgggaaaaaagaggccggtagagcactctcctgtggagccagactcctcctcgggaaccggaaaggcgggccagcagcctgcaagaaaaagattgaattttggtcagactggagacgcagactcagtacctgacccccagcctctcggacagccaccagcagccccctctggtctgggaactaatacgatggctacaggcagtggcgcaccaatggcagacaataacgagggcgccgacggagtgggtaattcctcgggaaattggcattgcgattccacatggatgggcgacagagtcatcaccaccagcacccgaacctgggccctgcccacctacaacaaccacctctacaaacaaatttccagccaatcaggagcctcgaacgacaatcactactttggctacagcaccccttgggggtattttgacttcaacagattccactgccacttttcaccacgtgactggcaaagactcatcaacaacaactggggattccgacccaagagactcaacttcaagctctttaacattcaagtcaaagaggtcacgcagaatgacggtacgacgacgattgccaataaccttaccagcacggttcaggtgtttactgactcggagtaccagctcccgtacgtcctcggctcggcgcatcaaggatgcctcccgccgttcccagcagacgtcttcatggtgccacagtatggatacctcaccctgaacaacgggagtcaggcagtaggacgctcttcattttactgcctggagtactttccttctcagatgctgcgtaccggaaacaactttaccttcagctacacttttgaggacgttcctttccacagcagctacgctcacagccagagtctggaccgtctcatgaatcctctcatcgaccagtacctgtattacttgagcagaacaaacactccaagtggaaccaccacgcagtcaaggcttcagttttctcaggccggagcgagtgacattcgggaccagtctaggaactggcttcctggaccctgttaccgccagcagcgagtatcaaagacatctgcggataacaacaacagtgaatactcgtggactggagctaccaagtaccacctcaatggcagagactctctggtgaatccgggcccggccatggcaagccacaaggacgatgaagaaaagttttttcctcagagcggggttctcatctttgggaagcaaggctcagagaaaacaaatgtggacattgaaaaggtcatgattacagacgaagaggaaatcaggacaaccaatcccgtggctacggagcagtatggttctgtatctaccaacctccagagaggcaacctagcaatctccgaccagacaaaacacgctaggcaagcagctaccgcagatgtcaacacacaaggcgttcttccaggcatggtctggcaggacagagatgtgtaccttcaggggcccatctgggcaaagattccacacacggacggacattttcacccctctcccctcatgggtggattcggacttaaacaccctcctccccagattctcatcaagaacaccccggtacctgcgaatccttcgaccaccttcagtgcggcaaagtttgcttccttcatcacacagtactccacgggacaggtcagcgtggagatcgagtgggagctgcagaaggaaaacagcaaacgctggaatcccgaaattcagtacacttccaactacaacaagtctattaatgtggactttactgtggacactaatggcgtgtattcagagcctcgccccattggcaccagatacctgactcgtaatctgtaa

SEQ ID NO: 4 - protein, 746 aa, synthetic construct
  REGION 1..746: note = synthetically generated sequence
MAADGYLPDWLEDTLSEGIRQWWKLKPGPPPPKPAERHKDDSRGLVLPGYKYLGPFNGLDKGEPVNEADAAALEHDKAYDRQLDSGDNPYLKYNHADAEFQERLKEDTSFGGNLGRAVFQAKKRVLEPLGLVEEPVKTAPGKKRPVEHSPVEPDSSSGTGKAGQQPARKRLNFGQTGDADSVPDPQPLGQPPAAPSGLGTNTMATGSGAPMADNNEGADGVGNSSGNWHCDSTWMGDRVITTSTRTWALPTYNNHLYKQISSQSGASNDNHYFGYSTPWGYFDFNRFHCHFSPRDWQRLINNNWGFRPKRLNFKLFNIQVKEVTQNDGTTTIANNLTSTVQVFTDSEYQLPYVLGSAHQGCLPPFPADVFMVPQYGYLTLNNGSQAVGRSSFYCLEYFPSQMLRTGNNFTFSYTFEDVPFHSSYAHSQSLDRLMNPLIDQYLYYLSRTNTPSGTTTQSRLQFSQAGASDIRDQSRNWLPGPCYRQQRVSKTSADNNNSEYSWTGATKYHLNGRDSLVNPGPAMASHKDDEEKFFPQSGVLIFGKQGSEKTNVDIEKVMITDEEEIRTTNPVATEQYGSVSTNLQRGNLAISDQTKHAARQAATADVNTQGVLPGMVWQDRDVYLQGPIWAKIPHTDGHFHPSPLMGGFGLKHPPPQILIKNTPVPANPSTTFSAAKFASFITQYSTGQVSVEIEWELQKENSKRWNPEIQYTSNYNKSINVDFTVDTNGVYSEPRPIGTRYLTRNL

SEQ ID NO: 5 - DNA, 2238 bp, synthetic construct
  misc_feature 1..2238: note = synthetically generated sequence
  source 1..2238: mol_type = other DNA
atggctgccgatggttatcttccagattggctcgaggacactctctctgaaggaataagacagtggtggaagctcaaacctggcccaccaccaccaaagcccgcagagcggcataaggacgacagcaggggtcttgtgcttcctgggtacaagtacctcggacccttcaacggactcgacaagggagagccggtcaacgaggcagacgccgcggccctcgagcacgacaaagcctacgaccggcagctcgacagcggagacaacccgtacctcaagtacaaccacgccgacgcggagtttcaggagcgccttaaagaagatacgtcttttgggggcaacctcggacgagcagtcttccaggcgaaaaagagggttcttgaacctctgggcctggttgaggaacctgttaagacggctccgggaaaaaagaggccggtagagcactctcctgtggagccagactcctcctcgggaaccggaaaggcgggccagcagcctgcaagaaaaagattgaattttggtcagactggagacgcagactcagtacctgacccccagcctctcggacagccaccagcagccccctctggtctgggaactaatacgatggctacaggcagtggcgcaccaatggcagacaataacgagggcgccgacggagtgggtaattcctcgggaaattggcattgcgattccacatggatgggcgacagagtcatcaccaccagcacccgaacctgggccctgcccacctacaacaaccacctctacaaacaaatttccagccaatcaggagcctcgaacgacaatcactactttggctacagcaccccttgggggtattttgacttcaacagattccactgccacttttcaccacgtgactggcaaagactcatcaacaacaactggggattccgacccaagagactcaacttcaagctctttaacattcaagtcaaagaggtcacgcagaatgacggtacgacgacgattgccaataaccttaccagcacggttcaggtgtttactgactcggagtaccagctcccgtacgtcctcggctcggcgcatcaaggatgcctcccgccgttcccagcagacgtcttcatggtgccacagtatggatacctcaccctgaacaacgggagtcaggcagtaggacgctcttcattttactgcctggagtactttccttctcagatgctgcgtaccggaaacaactttaccttcagctacacttttgaggacgttcctttccacagcagctacgctcacagccagagtctggaccgtctcatgaatcctctcatcgaccagtacctgtattacttgagcagaacaaacactccaagtggaaccaccacgcagtcaaggcttcagttttctcaggccggagcgagtgacattcgggaccagtctaggaactggcttcctggaccctgttaccgccagcagcgagtatcaaagacatctgcggataacaacaacagtgaatactcgtggactggagctaccaagtaccacctcaatggcagagactctctggtgaatccgggcccggccatggcaagccacaaggacgatgaagaaaagttttttcctcagagcggggttctcatctttgggaagcaaggctcagagaaaacaaatgtggacattgaaaaggtcatgattacaaacgaagaggaaatcagggcaaccaatcccgtggctacggagcagtatggttctgtatctaccaacctccagagaggcaacctagcaatctccgaccagacaaaacacgctaggcaagcagctaccgcagatgtcaacacacaaggcgttcttccaggcatggtctggcaggacagagatgtgtaccttcaggggcccatctgggcaaagattccacacacggacggacattttcacccctctcccctcatgggtggattcggacttaaacaccctcctccccagattctcatcaagaacaccccggtacctgcgaatccttcgaccaccttcagtgcggcaaagtttgcttccttcatcacacagtactccacgggacaggtcagcgtggagatcgagtgggagctgcagaaggaaaacagcaaacgctggaatcccgaaattcagtacacttccaactacaacaagtctattaatgtggactttactgtggacactaatggcgtgtattcagagcctcgccccattggcaccagatacctgactcgtaatctgtaa

SEQ ID NO: 6 - protein, 746 aa, synthetic construct
  REGION 1..746: note = synthetically generated sequence
MAADGYLPDWLEDTLSEGIRQWWKLKPGPPPPKPAERHKDDSRGLVLPGYKYLGPFNGPDKGEPVNEADAAALEHDKAYDRQLDSGDNPYLKYNHADAEFQERLKEDTSFGGNLGRAVFQAKKRVLEPLGLVEEPVKTAPGKKRPVEHSPVEPDSSSGTGKAGQQPARKRLNFGQTGDADSVPDPQPLGQPPAAPSGLGTNTMATGSGAPMADNNEGADGVGNSSGNWHCDSTWMGDRVITTSTRTWALPTYNNHLYKQISSQSGASNDNHYFGYSTPWGYFDFNRFHCHFSPRDWQRLINNNWGFRPKRLNFKLFNIQVKEVTQNDGTTTIANNLTSTVQVFTDSEYQLPYVLGSAHQGCLPPFPADVFMVPQYGYLTLNNGSQAVGRSSFYCLEYFPSQMLRTGNNFTFSYTFEDVPFHSSYAHSQSLDRLMNPLIDQYLYYLSRTNTPSGTTTQSRLQFSQAGASDIRDQSRNWLPGPCYRQQRVSKTSADNDNSEYSWTGATKYHLNGRDSLVNPGPAMASHKDDEEKFFPQSGVLIFGKQGSEKTNVDIEKVMITDEEEIRATNPVATEQYGSVSTNLQRGNLAISDQTKHAARQAATADVNTQGVLPGMVWQDRDVYLQGPIWAKIPHTDGHFHPSPLMGGFGLKHPPPQILIKNTPVPANPSTTFSAAKFASFITQYSTGQVSVEIEWELQKENSKRWNPEIQYTSNYNKSINVDFTVDTNGVYSEPRPIGTRYLTRNL

SEQ ID NO: 7 - DNA, 2238 bp, synthetic construct
  misc_feature 1..2238: note = synthetically generated sequence
  source 1..2238: mol_type = other DNA
atggctgccgatggttatcttccagattggctcgaggacactctctctgaaggaataagacagtggtggaagctcaaacctggcccaccaccaccaaagcccgcagagcggcataaggacgacagcaggggtcttgtgcttcctgggtacaagtacctcggacccttcaacggactcgacaagggagagccggtcaacgaggcagacgccgcggccctcgagcacgacaaagcctacgaccggcagctcgacagcggagacaacccgtacctcaagtacaaccacgccgacgcggagtttcaggagcgccttaaagaagatacgtcttttgggggcaacctcggacgagcagtcttccaggcgaaaaagagggttcttgaacctctgggcctggttgaggaacctgttaagacggctccgggaaaaaagaggccggtagagcactctcctgtggagccagactcctcctcgggaaccggaaaggcgggccagcagcctgcaagaaaaagattgaattttggtcagactggagacgcagactcagtacctgacccccagcctctcggacagccaccagcagccccctctggtctgggaactaatacgatggctacaggcagtggcgcaccaatggcagacaataacgagggcgccgacggagtgggtaattcctcgggaaattggcattgcgattccacatggatgggcgacagagtcatcaccaccagcacccgaacctgggccctgcccacctacaacaaccacctctacaaacaaatttccagccaatcaggagcctcgaacgacaatcactactttggctacagcaccccttgggggtattttgacttcaacagattccactgccacttttcaccacgtgactggcaaagactcatcaacaacaactggggattccgacccaagagactcaacttcaagctctttaacattcaagtcaaagaggtcacgcagaatgacggtacgacgacgattgccaataaccttaccagcacggttcaggtgtttactgactcggagtaccagctcccgtacgtcctcggctcggcgcatcaaggatgcctcccgccgttcccagcagacgtcttcatggtgccacagtatggatacctcaccctgaacaacgggagtcaggcagtaggacgctcttcattttactgcctggagtactttccttctcagatgctgcgtaccggaaacagctttaccttcagctacacttttgaggacgttcctttccacagcagctacgctcacagccagagtctggaccgtctcatgaatcctctcatcgaccagtacctgtattacttgagcagaacaaacactccaagtggaaccaccacgcagtcaaggcttcagttttctcaggccggagcgagtgacattcgggaccagtctaggaactggcttcctggaccctgttaccgccagcagcgagtatcaaagacatctgcggataacaacaacagtgaatactcgtggactggagctaccaagtaccacctcaatggcagagactctctggtgaatccgggcccggccatggcaagccacaaggacgatgaagaaaagttttttcctcagagcggggttctcatctttgggaagcaaggctcagagaaaacaaatgtggacattgaaaaggtcatgattacagacgaagaggaaatcaggacaaccaatcccgtggctacggagcagtatggttctgtatctaccaacctccagagaggcaacctagcaaaggatcagacaaaaagcaccgctaggcaagcagctaccgcagatgtcaacacacaaggcgttcttccaggcatggtctggcaggacagagatgtgtaccttcaggggcccatctgggcaaagattccacacacggacggacattttcacccctctcccctcatgggtggattcggacttaaacaccctcctccccagattctcatcaagaacaccccggtacctgcgaatccttcgaccaccttcagtgcggcaaagtttgcttccttcatcacacagtactccacgggacaggtcagcgtggagatcgagtgggagctgcagaaggaaaacagcaaacgctggaatcccgaaattcagtacacttccaactacaacaagtctattaatgtggactttactgtggacactaatggcgtgtattcagagcctcgccccattggcaccagatacctgactcgtaatctgtaa

SEQ ID NO: 8 - protein, 745 aa, synthetic construct
  REGION 1..745: note = synthetically generated sequence
MAADGYLPDWLEDTLSEGIRQWWKLKPGPPPPKPAERHKDDSRGLVLPGYKYLGPFNGLDKGEPVNEADAAALEHDKAYDRQLDSGDNPYLKYNHADAEFQERLKEDTSFGGNLGRAVFQAKKRVLEPLGLVEEPVKTAPGKKRPVEHSPVEPDSSSGTGKAGQQPARKRLNFGQTGDADSVPDPQPLGQPPAAPSGLGTNTMATGSGAPMADNNEGADGVGNSSGNWHCDSTWMGDRVITTSTRTWALPTYNNHLYKQISSQSGASNDNHYFGYSTPWGYFDFNRFHCHFSPRDWQRLINNNWGFRPKRLNFKLFNIQVKEVTQNDGTTTIANNLTSTVQVFTDSEYQLPYVLGSAHQGCLPPFPADVFMVPQYGYLTLNNGSQAVGRSSFYCLEYFPSQMLRTGNSFTFSYTFEDVPFHSSYAHSQSLDRLMNPLIDQYLYYLSRTNTPSGTTTQSRLQFSQAGASDIRDQSRNWLPGPCYRQQRVSKTSADNNNSEYSWTGATKYHLNGRDSLVNPGPAMASHKDDEEKFFPQSGVLIFGKQGSEKTNVDIEKVMITDEEEIRTTNPVATEQYGSVSTNLQRGNLAKDQTKSTARQAATADVNTQGVLPGMVWQDRDVYLQGPIWAKIPHTDGHFHPSPLMGGFGLKHPPPQILIKNTPVPANPSTTFSAAKFASFITQYSTGQVSVEIEWELQKENSKRWNPEIQYTSNYNKSINVDFTVDTNGVYSEPRPIGTRYLTRNL

SEQ ID NO: 9 - DNA, 2238 bp, synthetic construct
  misc_feature 1..2238: note = synthetically generated sequence
  source 1..2238: mol_type = other DNA
atggctgccgatggttatcttccagattggctcgaggacactctctctgaaggaataagacagtggtggaagctcaaacctggcccaccaccaccaaagcccgcagagcggcataaggacgacagcaggggtcttgtgcttcctgggtacaagtacctcggacccttcaacggactcgacaagggagagccggtcaacgaggcagacgccgcggccctcgagcacgacaaagcctacgaccggcagctcgacagcggagacaacccgtacctcaagtacaaccacgccgacgcggagtttcaggagcgccttaaagaagatacgtcttttgggggcaacctcggacgagcagtcttccaggcgaaaaagagggttcttgaacctctgggcctggttgaggaacctgttaagacggctccgggaaaaaagaggccggtagagcactctcctgtggagccagactcctcctcgggaaccggaaaggcgggccagcagcctgcaagaaaaagattgaattttggtcagactggagacgcagactcagtacctgacccccagcctctcggacagccaccagcagccccctctggtctgggaactaatacgatggctacaggcagtggcgcaccaatggcagacaataacgagggcgccgacggagtgggtaattcctcgggaaattggcattgcgattccacatggatgggcgacagagtcatcaccaccagcacccgaacctgggccctgcccacctacaacaaccacctctacaaacaaatttccagccaatcaggagcctcgaacgacaatcactactttggctacagcaccccttgggggtattttgacttcaacagattccactgccacttttcaccacgtgactggcaaagactcatcaacaacaactggggattccgacccaagagactcaacttcaagctctttaacattcaagtcaaagaggtcacgcagaatgacggtacgacgacgattgccaataaccttaccagcacggttcaggtgtttactgactcggagtaccagctcccgtacgtcctcggctcggcgcatcaaggatgcctcccgccgttcccagcagacgtcttcatggtgccacagtatggatacctcaccctgaacaacgggagtcaggcagtaggacgctcttcattttactgcctggagtactttccttctcagatgctgcgtaccggaaacaactttaccttcagctacacttttgaggacgttcctttccacagcagctacgctcacagccagagtctggaccgtctcatgaatcctctcatcgaccagtacctgtattacttgagcagaacaaacactccaagtggaaccaccacgcagtcaaggcttcagttttctcaggccggagcgagtgacattcgggaccagtctaggaactggcttcctggaccctgttaccgccagcagcgagtatcaaagacacctgcggataacaacaacagtgaatactcgtggactggagctaccaagtaccacctcaatggcagagactctctggtgaatccgggcccggccatggcaagccacaaggacgatgaagaaaagttttttcctcagagcggggttctcatctttgggaagcaaggctcagagaaaacaaatgtggacattgaaaaggtcatgattacagacgaagaggaaatcaggacaaccaatcccgtggctacggagcagtatggttctgtatctaccaacctccagagaggcaacctagcaaaccaagactacacaaaaactgctaggcaagcagctaccgcagatgtcaacacacaaggcgttcttccaggcatggtctggcaggacagagatgtgtaccttcaggggcccatctgggcaaagattccacacacggacggacattttcacccctctcccctcatgggtggattcggacttaaacaccctcctccccagattctcatcaagaacaccccggtacctgcgaatccttcgaccaccttcagtgcggcaaagtttgcttccttcatcacacagtactccacgggacaggtcagcgtggagatcgagtgggagctgcagaaggaaaacagcaaacgctggaatcccgaaattcagtacacttccaactacaacaagtctgttaatgtggactttactgtggacactaatggcgtgtattcagagcctcgccccattggcaccagatacctgactcgtaatctgtaa

SEQ ID NO: 10 - protein, 745 aa, synthetic construct
  REGION 1..745: note = synthetically generated sequence
MAADGYLPDWLEDTLSEGIRQWWKLKPGPPPPKPAERHKDDSRGLVLPGYKYLGPFNGLDKGEPVNEADAAALEHDKAYDRQLDSGDNPYLKYNHADAEFQERLKEDTSFGGNLGRAVFQAKKRVLEPLGLVEEPVKTAPGKKRPVEHSPVEPDSSSGTGKAGQQPARKRLNFGQTGDADSVPDPQPLGQPPAAPSGLGTNTMATGSGAPMADNNEGADGVGNSSGNWHCDSTWMGDRVITTSTRTWALPTYNNHLYKQISSQSGASNDNHYFGYSTPWGYFDFNRFHCHFSPRDWQRLINNNWGFRPKRLNFKLFNIQVKEVTQNDGTTTIANNLTSTVQVFTDSEYQLPYVLGSAHQGCLPPFPADVFMVPQYGYLTLNNGSQAVGRSSFYCLEYFPSQMLRTGNNFTFSYTFEDVPFHSSYAHSQSLDRLMNPLIDQYLYYLSRTNTPSGTTTQSRLQFSQAGASDIRDQSRNWLPGPCYRQQRVSKTPADNNNSEYSWTGATKYHLNGRDSLVNPGPAMASHKDDEEKFFPQSGVLIFGKQGSEKTNVDIEKVMITDEEEIRTTNPVATEQYGSVSTNLQRGNLANQDYTKTARQAATADVNTQGVLPGMVWQDRDVYLQGPIWAKIPHTDGHFHPSPLMGGFGLKHPPPQILIKNTPVPANPSTTFSAAKFASFITQYSTGQVSVEIEWELQKENSKRWNPEVQYTSNYNKSINVDFTVDTNGVYSEPRPIGTRYLTRNL

SEQ ID NO: 11 - DNA, 2238 bp, synthetic construct
  misc_feature 1..2238: note = synthetically generated sequence
  source 1..2238: mol_type = other DNA
atggctgccgatggttatcttccagattggctcgaggacactctctctgaaggaataagacagtggtggaagctcaaacctggcccaccaccaccaaagcccgcagagcggcataaggacgacagcaggggtcttgtgcttcctgggtacaagtacctcggacccttcaacggactcgacaagggagagccggtcaacgaggcagacgccgcggccctcgagcacgacaaagcctacgaccggcagctcgacagcggagacaacccgtacctcaagtacaaccacgccgacgcggagtttcaggagcgccttaaagaagatacgtcttttgggggcaacctcggacgagcagtcttccaggcgaaaaagagggttcttgaacctctgggcctggttgaggaacctgttaagacggctccgggaaaaaagaggccggtagagcactctcctgtggagccagactcctcctcgggaaccggaaaggcgggccagcagcctgcaagaaaaagattgaattttggtcagactggagacgcagactcagtacctgacccccagcctctcggacagccaccagcagccccctctggtctgggaactaatacgatggctacaggcagtggcgcaccaatggcagacaataacgagggcgccgacggagtgggtaattcctcgggaaattggcattgcgattccacatggatgggcgacagagtcatcaccaccagcacccgaacctgggccctgcccacctacaacaaccacctctacaaacaaatttccagccaatcaggagcctcgaacgacaatcactactttggctacagcaccccttgggggtattttgacttcaacagattccactgccacttttcaccacgtgactggcaaagactcatcaacaacaactggggattccgacccaagagactcaacttcaagctctttaacattcaagtcaaagaggtcacgcagaatgacggtacgacgacgattgccaataaccttaccagcacggttcaggtgtttactgactcggagtaccagctcccgtacgtcctcggctcggcgcatcaaggatgcctcccgccgttcccagcagacgtcttcatggtgccacagtatggatacctcaccctgaacaacgggagtcaggcagtaggacgctcttcattttactgcctggagtactttccttctcagatgctgcgtaccggaaacaactttaccttcagctacacttttgaggacgttcctttccacagcagctacgctcacagccagagtctggaccgtctcatgaatcctctcatcgaccagtacctgtattacttgagcagaacaaacactccaagtggaaccaccacgcagtcaaggcttcagttttctcaggccggagcgagtgacattcgggaccagtctaggaactggcttcctggaccctgttaccgccagcagcgagtatcaaagacatatgcggataacaacaacagtgaatactcgtggactggagctaccaagtaccacctcaatggcagagactctctggtgaatccgggcccggccatggcaagccacaaggacgatgaagaaaagttttttcctcagagcggggttctcatctttgggaagcaaggctcagagaaaacaaatgtggacattgaaaaggtcatgattacagacgaagaggaaatcaggacaaccaatcccgtggctacggagcagtatggttctgtatctaccaacctccagagaggcaacctagcaatctccgaccagacaaaacacgctaggcaagcagctaccgcagatgtcaacacacaaggcgttcttccaggcatggtctggcaggacagagatgtgtaccttcaggggcccatctgggcaaagattccacacacggacggacattttcacccctctcccctcatgggtggattcggacttaaacaccctcctccccagattctcatcaagaacaccccggtacctgcgaatccttcgaccaccttcagtgcggcaaagtttgcttccttcatcacacagtactccacgggacaggtcagcgtggagatcgagtgggagctgcagaaggaaaacagcaaacgctggaatcccgaaattcagtacacttccaactacaacaagtctattaatgtggactttactgtggacactaatggcgtgtattcagagcctcgccccattggcaccagatacctgactcgtaatctgtaa

SEQ ID NO: 12 - protein, 745 aa, synthetic construct
  REGION 1..745: note = synthetically generated sequence
MAADGYLPDWLEDTLSEGIRQWWKLKPGPPPPKPAERHKDDSRGLVLPGYKYLGPFNGLDKGEPVNEADAAALEHDKAYDRQLDSGDNPYLKYNHADAEFQERLKEDTSFGGNLGRAVFQAKKRVLEPLGLVEEPVKTAPGKKRPVEHSPVEPDSSSGTGKAGQQPARKRLNFGQTGDADSVPDPQPLGQPPAAPSGLGTNTMATGSGAPMADNNEGADGVGNSSGNWHCDSTWMGDRVITTSTRTWALPTYNNHLYKQISSQSGASNDNHYFGYSTPWGYFDFNRFHCHFSPRDWQRLINNNWGFRPKRLNFKLFNIQVKEVTQNDGTTTIANNLTSTVQVFTDSEYQLPYVLGSAHQGCLPPFPADVFMVPQYGYLTLNNGSQAVGRSSFYCLEYFPSQMLRTGNNFTFSYTFEDVPFHSSYAHSQSLDRLMNPLIDQYLYYLSRTNTPSGTTTQSRLQFSQAGASDIRDQSRNWLPGPCYRQQRVSKTYADNNNSEYSWTGATKYHLNGRDSLVNPGPAMASHKDDEEKFFPQSGVLIFGKQGSEKTNVDIEKVMITDEEEIRTTNPVATEQYGSVSTNLQRGNLAISDQTKHARQAATADVNTQGVLPGMVWQDRDVYLQGPIWAKIPHTDGHFHPSPLMGGFGLKHPPPQILIKNTPVPANPSTTFSAAKFASFITQYSTGQVSVEIEWELQKENSKRWNPEIQYTSNYNKSINVDFTVDTNGVYSEPRPIGTRYLTRNL

SEQ ID NO: 13 - DNA, 2238 bp, synthetic construct
  misc_feature 1..2238: note = synthetically generated sequence
  source 1..2238: mol_type = other DNA
atggctgccgatggttatcttccagattggctcgaggacactctctctgaaggaataagacagtggtggaagctcaaacctggcccaccaccaccaaagcccgcagggcggcataaggacgacagcaggggtcttgtgcttcctgggtacaagtacctcggacccttcaacggactcgacaagggagagccggtcaacgaggcagacgccgcggccctcgagcacgacaaagcctacgaccggcagctcgacagcggagacaacccgtacctcaagtacaaccacgccgacgcggagtttcaggagcgccttaaagaagatacgtcttttgggggcaacctcggacgagcagtcttccaggcgaaaaagagggttcttgaacctctgggcctggttgaggaacctgttaagacggctccgggaaaaaagaggccggtagagcactctcctgtggagccagactcctcctcgggaaccggaaaggcgggccagcagcctgcaagaaaaagattgaattttggtcagactggagacgcagactcagtacctgacccccagcctctcggacagccaccagcagccccctctggtctgggaactaatacgatggctacaggcagtggcgcaccaatggcagacaataacgagggcgccgacggagtgggtaattcctcgggaaattggcattgcgattccacatggatgggcgacagagtcatcaccaccagcacccgaacctgggccctgcccacctacaacaaccacctctacaaacaaatttccagccaatcaggagcctcgaacgacaatcactactttggctacagcaccccttgggggtattttgacttcaacagattccactgccacttttcaccacgtgactggcaaagactcatcaacaacaactggggattccgacccaagagactcaacttcaagctctttaacattcaagtcaaagaggtcacgcagaatgacggtacgacgacgattgccaataaccttaccagcacggttcaggtgtttactgactcggagtaccagctcccgtacgtcctcggctcggcgcatcaaggatgcctcccgccgttcccagcagacgtcttcatggtgccacagtatggatacctcaccctgaacaacgggagtcaggcagtaggacgctcttcattttactgcctggagtactttccttctcagatgctgcgtaccggaaacaactttaccttcagctacacttttgaggacgttcctttccacagcagctacgctcacagccagagtctggaccgtctcatgaatcctctcatcgaccagtacctgtattacttgagcagaacaaacactccaagtggaaccaccacgcagtcaaggcttcagttttctcaggccggagcgagtgacattcgggaccagtctaggaactggcttcctggaccctgttaccgccagcagcgagtatcaaagacatctgcggataacaacaacagtgaatactcgtggactggagctaccaagtaccacctcaatggcagagactctctggtgaatccgggcccggccatggcaagccacaaggacgatgaagaaaagttttttcctcagagcggggttctcatctttgggaagcaaggctcagagaaaacaaatgtggacattgaaaaggtcatgattacagacgaagaggaaatcaggacaaccaatcccgtggctacggagcagtatggttctgtatctaccaacctccagagaggcaacctagcaaaccaagactacacaaaaactgctaggcaagcagctaccgcagatgtcaacacacaaggcgttcttccaggcatggtctggcaggacagagatgtgtaccttcaggggcccatctgggcaaagattccacacacggacggacattttcacccctctcccctcatgggtggattcggacttaaacaccctcctccccagattctcatcaagaacaccccggtacctgcgaatccttcgaccaccttcagtgcggcaaagtttgcttccttcatcacacagtactccacgggacaggtcagcgtggagatcgagtgggagctgcagaaggaaaacagcaaacgctggaatcccgaaattcagtacacttccaactacaacaagtctattaatgtggactttactgtggacactaatggcgtgtattcagagcctcgccccattggcaccagatacctgactcgtaatctgtaa

SEQ ID NO: 14 - protein, 745 aa, synthetic construct
  REGION 1..745: note = synthetically generated sequence
MAADGYLPDWLEDTLSEGIRQWWKLKPGPPPPKPAGRHKDDSRGLVLPGYKYLGPFNGLDKGEPVNEADAAALEHDKAYDRQLDSGDNPYLKYNHADAEFQERLKEDTSFGGNLGRAVFQAKKRVLEPLGLVEEPVKTAPGKKRPVEHSPVEPDSSSGTGKAGQQPARKRLNFGQTGDADSVPDPQPLGQPPAAPSGLGTNTMATGSGAPMADNNEGADGVGNSSGNWHCDSTWMGDRVITTSTRTWALPTYNNHLYKQISSQSGASNDNHYFGYSTPWGYFDFNRFHCHFSPRDWQRLINNNWGFRPKRLNFKLFNIQVKEVTQNDGTTTIANNLTSTVQVFTDSEYQLPYVLGSAHQGCLPPFPADVFMVPQYGYLTLNNGSQAVGRSSFYCLEYFPSQMLRTGNNFTFSYTFEDVPFHSSYAHSQSLDRLMNPLIDQYLYYLSRTNTPSGTTTQSRLQFSQAGASDIRDQSRNWLPGPCYRQQRVSKTSADNNNSEYSWTGATKYHLNGRDSLVNPGPAMASHKDDEEKFFPQSGVLIFGKQGSEKTNVDIEKVMITDEEEIRTTNPVATEQYGSVSTNLQRGNLANQDYTKTARQAATADVNTQGVLPGMVWQDRDVYLQGPIWAKIPHTDGHFHPSPLMGGFGLKHPPPQILIKNTPVPANPSTTFSAAKFASFITQYSTGQVSVEIEWELQKENSKRWNPEIQYTSNYNKSINVDFTVDTNGVYSEPRPIGTRYLTRNL

SEQ ID NO: 15 - DNA, 2238 bp, synthetic construct; identical to SEQ ID NO: 3
  misc_feature 1..2238: note = synthetically generated sequence
  source 1..2238: mol_type = other DNA

SEQ ID NO: 16 - protein, 745 aa, synthetic construct
  REGION 1..745: note = synthetically generated sequence
MAADGYLPDWLEDTLSEGIRQWWKLKPGPPPPKPAERHKDDSRGLVLPGYKYLGPFNGLDKGEPVNEADAAALEHDKAYDRQLDSGDNPYLKYNHADAEFQERLKEDTSFGGNLGRAVFQAKKRVLEPLGLVEEPVKTAPGKKRPVEHSPVEPDSSSGTGKAGQQPARKRLNFGQTGDADSVPDPQPLGQPPAAPSGLGTNTMATGSGAPMADNNEGADGVGNSSGNWHCDSTWMGDRVITTSTRTWALPTYNNHLYKQISSQSGASNDNHYFGYSTPWGYFDFNRFHCHFSPRDWQRLINNNWGFRPKRLNFKLFNIQVKEVTQNDGTTTIANNLTSTVQVFTDSEYQLPYVLGSAHQGCLPPFPADVFMVPQYGYLTLNNGSQAVGRSSFYCLEYFPSQMLRTGNNFTFSYTFEDVPFHSSYAHSQSLDRLMNPLIDQYLYYLSRTNTPSGTTTQSRLQFSQAGASDIRDQSRNWLPGPCYRQQRVSKTSADNNNSEYSWTGATKYHLNGRDSLVNPGPAMASHKDDEEKFFPQSGVLIFGKQGSEKTNVDIEKVMITDEEEIRTTNPVATEQYGSVSTNLQRGNLAISDQTKHARQAATADVNTQGVLPGMVWQDRDVYLQGPIWAKIPHTDGHFHPSPLMGGFGLKHPPPQILIKNTPVPANPSTTFSAAKFASFITQYSTGQVSVEIEWELQKENSKRWNPEIQYTSNYNKSINVDFTVDTNGVYSEPRPIGTRYLTRNL

SEQ ID NO: 17 - DNA, 2238 bp, synthetic construct
  misc_feature 1..2238: note = synthetically generated sequence
  source 1..2238: mol_type = other DNA
atggctgccgatggttatcttccagattggctcgaggacactctctctgaaggaataagacagtggtggaagctcaaacctggcccaccaccaccaaagcccgcagagcggcataaggacgacagcaggggtcttgtgcttcctgggtacaagtacctcggacccttcaacggactcgacaagggagagccggtcaacgaggcagacgccgcggccctcgagcacgacaaagcctacgaccggcagctcgacagcggagacaacccgtacctcaagtacaaccacgccgacgcggagtttcaggagcgccttaaagaagatacgtcttttgggggcaacctcggacgagcagtcttccaggcgaaaaagagggttcttgaacctctgggcctggttgaggaacctgttaagacggctccgggaaaaaagaggccggtagagcactctcctgtggagccagactcctcctcgggaaccggaaaggcgggccagcagcctgcaagaaaaagattgaattttggtcagactggagacgcagactcagtacctgacccccagcctctcggacagccaccagcagccccctctggtctgggaactaatacgatggctacaggcagtggcgcaccaatggcagacaataacgagggcgccgacggagtgggtaattcctcgggaaattggcattgcgattccacatggatgggcgacagagtcatcaccaccagcacccgaacctgggccctgcccacctacaacaaccacctctacaaacaaatttccagccaatcaggagcctcgaacgacaatcactactttggctacagcaccccttgggggtattttgacttcaacagattccactgccacttttcaccacgtgactggcaaagactcatcaacaacaactggggattccgacccaagagactcaacttcaagctctttaacattcaagtcaaagaggtcacgcagaatgacggtacgacgacgattgccaataaccttaccagcacggttcaggtgtttactgactcggagtaccagctcccgtacgtcctcggctcggcgcatcaaggatgcctcccgccgttcccagcagacgtcttcatggtgccacagtatggatacctcaccctgaacaacgggagtcaggcagtaggacgctcttcattttactgcctggagtactttccttctcagatgctgcgtaccggaaacagctttaccttcagctacacttttgaggacgttcctttccacagcagctacgctcacagccagagtctggaccgtctcatgaatcctctcatcgaccagtacctgtattacttgagcagaacaaacactccaagtggaaccaccacgcagtcaaggcttcagttttctcaggccggagcgagtgacattcgggaccagtctaggaactggcttcctggaccctgttaccgccagcagcgagtatcaaagacatctgcggataacaacaacagtgaatactcgtggactggagctaccaagtaccacctcaatggcagagactctctggtgaatccgggcccggccatggcaagccacaaggacgatgaagaaaagttttttcctcagagcggggttctcatctttgggaagcaaggctcagagaaaacaaatgtggacattgaaaaggtcatgattacagacgaagaggaaatcaggacaaccaatcccgtggctacggagcagtatggttctgtatctaccaacctccagagaggcaacctagcacacgacatcaccaagaatattgctaggcaagcagctaccgcagatgtcaacacacaaggcgttcttccaggcatggtctggcaggacagagatgtgtaccttcaggggcccatctgggcaaagattccacacacggacggacattttcacccctctcccctcatgggtggattcggacttaaacaccctcctccccagattctcatcaagaacaccccggtacctgcgaatccttcgaccaccttcagtgcggcaaagtttgcttccttcatcacacagtactccacgggacaggtcagcgtggagatcgagtgggagctgcagaaggaaaacagcaaacgctggaatcccgaaattcagtacacttccaactacaacaagtctattaatgtggactttactgtggacactaatggcgtgtattcagagcctcgccccattggcaccagatacctgactcgtaatctgtaa

SEQ ID NO: 18 - protein, 745 aa, synthetic construct
  REGION 1..745: note = synthetically generated sequence
MAADGYLPDWLEDTLSEGIRQWWKLKPGPPPPKPAERHKDDSRGLVLPGYKYLGPFNGLDKGEPVNEADAAALEHDKAYDRQLDSGDNPYLKYNHADAEFQERLKEDTSFGGNLGRAVFQAKKRVLEPLGLVEEPVKTAPGKKRPVEHSPVEPDSSSGTGKAGQQPARKRLNFGQTGDADSVPDPQPLGQPPAAPSGLGTNTMATGSGAPMADNNEGADGVGNSSGNWHCDSTWMGDRVITTSTRTWALPTYNNHLYKQISSQSGASNDNHYFGYSTPWGYFDFNRFHCHFSPRDWQRLINNNWGFRPKRLNFKLFNIQVKEVTQNDGTTTIANNLTSTVQVFTDSEYQLPYVLGSAHQGCLPPFPADVFMVPQYGYLTLNNGSQAVGRSSFYCLEYFPSQMLRTGNSFTFSYTFEDVPFHSSYAHSQSLDRLMNPLIDQYLYYLSRTNTPSGTTTQSRLQFSQAGASDIRDQSRNWLPGPCYRQQRVSKTSADNNNSEYSWTGATKYHLNGRDSLVNPGPAMASHKDDEEKFFPQSGVLIFGKQGSEKTNVDIEKVMITDEEEIRTTNPVATEQYGSVSTNLQRGNLAHDITKNIARQAATADVNTQGVLPGMVWQDRDVYLQGPIWAKIPHTDGHFHPSPLMGGFGLKHPPPQILIKNTPVPANPSTTFSAAKFASFITQYSTGQVSVEIEWELQKENSKRWNPEIQYTSNYNKSINVDFTVDTNGVYSEPRPIGTRYLTRNL

SEQ ID NO: 19 - DNA, 2238 bp, synthetic construct; identical to SEQ ID NO: 17
  misc_feature 1..2238: note = synthetically generated sequence
  source 1..2238: mol_type = other DNA

SEQ ID NO: 20 - protein, 745 aa, synthetic construct; identical to SEQ ID NO: 18
  REGION 1..745: note = synthetically generated sequence

SEQ ID NO: 21 - DNA, 2238 bp, synthetic construct
  misc_feature 1..2238: note = synthetically generated sequence
  source 1..2238: mol_type = other DNA
atggctgccgatggttatcttccagattggctcgaggacactctctctgaaggaataagacagtggtggaagctcaaacctggcccaccaccaccaaagcccgcagagcggcataaggacgacagcaggggtcttgtgcttcctgggtacaagtacctcggacccttcaacggactcgacaagggagagccggtcaacgacgcagacgccgcggccctcgagcacgacaaagcctacgaccggcagctcgacagcggagacaacccgtacctcaagtacaaccacgccgacgcggagtttcaggagcgccttaaagaagatacgtcttttgggggcaacctcggacgagcagtcttccaggcgaaaaagagggttcttgaacctctgggcctggttgaggaacctgttaagacggctccgggaaaaaagaggccggtagagcactctcctgtggagccagactcctcctcgggaaccggaaaggcgggccagcagcctgcaagaaaaagattgaattttggtcagactggagacgcagactcagtacctgacccccagcctctcggacagccaccagcagccccctctggtctgggaactaatacgatggctacaggcggtggcgcaccaatggcagacaataacgagggcgccgacggagtgggtaattcctcgggaaattggcattgcgattccacatggatgggcgacagagtcatcaccaccagcacccgaacctgggccctgcccacctacaacaaccacctctacaaacaaatttccagccaatcaggagcctcgaacgacaatcactactttggctacagcaccccttgggggtattttgacttcaacagattccactgccacttttcaccacgtgactggcaaagactcatcaacaacaactggggattccgacccaagagactcaacttcaagctctttaacattcaagtcaaagaggtcacgcagaatgacggtacgacgacgattgccaataaccttaccagcacggttcaggtgtttactgactcggagtaccagctcccgtacgtcctcggctcggcgcatcaaggatgcctcccgccgttcccagcagacgtcttcatggtgccacagtatggatacctcaccctgaacaacgggagtcaggcagtaggacgctcttcattttactgcctggagtactttccttctcagatgctgcgtaccggaaacagctttaccttcagctacacttttgaggacgttcctttccacagcagctacgctcacagccagagtctggaccgtctcatgaatcctctcatcgaccagtacctgtattacttgagcagaacaaacactccaagtggaaccaccacgcagtcaaggcttcagttttctcaggccggagcgagtgacattcgggaccagtctaggaactggcttcctggaccctgttaccgccagcagcgagtatcaaagacatctgcggataacaacaacagtgaatactcgtggactggagctaccaagtaccacctcaatggcagagactctctggtgaatccgggcccggccatggcaagccacaaggacgatgaagaaaagttttttcctcagagcggggttctcatctttgggaagcaaggctcagagaaaacaaatgtggacattgaaaaggtcatgattacagacgaagaggaaatcaggacaaccaatcccgtggctacggagcagtatggttctgtatctaccaacctccagagaggcaacctagcacacgacatcaccaagaatattgctaggcaagcagctaccgcagatgtcaacacacaaggcgttcttccaggcatggtctggcaggacagagatgtgtaccttcaggggcccatctgggcaaagattccacacacggacggacattttcacccctctcccctcatgggtggattcggacttaaacaccctcctccccagattctcatcaagaacaccccggtacctgcgaatccttcgaccaccttcagtgcggcaaagtttgcttccttcatcacacagtactccacgggacaggtcagcgtggagatcgagtgggagctgcagaaggaaaacagcaaacgctggaatcccgaaattcagtacacttccaactacaacaagtctattaatgtggactttactgtggacactaatggcgtgtattcagagcctcgccccattggcaccagatacctgactcgtaatctgtaa

SEQ ID NO: 22 - protein, 745 aa, synthetic construct
  REGION 1..745: note = synthetically generated sequence
MAADGYLPDWLEDTLSEGIRQWWKLKPGPPPPKPAERHKDDSRGLVLPGYKYLGPFNGLDKGEPVNDADAAALEHDKAYDRQLDSGDNPYLKYNHADAEFQERLKEDTSFGGNLGRAVFQAKKRVLEPLGLVEEPVKTAPGKKRPVEHSPVEPDSSSGTGKAGQQPARKRLNFGQTGDADSVPDPQPLGQPPAAPSGLGTNTMATGGGAPMADNNEGADGVGNSSGNWHCDSTWMGDRVITTSTRTWALPTYNNHLYKQISSQSGASNDNHYFGYSTPWGYFDFNRFHCHFSPRDWQRLINNNWGFRPKRLNFKLFNIQVKEVTQNDGTTTIANNLTSTVQVFTDSEYQLPYVLGSAHQGCLPPFPADVFMVPQYGYLTLNNGSQAVGRSSFYCLEYFPSQMLRTGNSFTFSYTFEDVPFHSSYAHSQSLDRLMNPLIDQYLYYLSRTNTPSGTTTQSRLQFSQAGASDIRDQSRNWLPGPCYRQQRVSKTSADNNNSEYSWTGATKYHLNGRDSLVNPGPAMASHKDDEEKFFPQSGVLIFGKQGSEKTNVDIEKVMITDEEEIRTTNPVATEQYGSVSTNLQRGNLAHDITKNIARQAATADVNTQGVLPGMVWQDRDVYLQGPIWAKIPHTDGHFHPSPLMGGFGLKHPPPQILIKNTPVPANPSTTFSAAKFASFITQYSTGQVSVEIEWELQKENSKRWNPEIQYTSNYNKSINVDFTVDTNGVYSEPRPIGTRYLTRNL

SEQ ID NO: 23 - DNA, 2238 bp, synthetic construct; identical to SEQ ID NO: 17
  misc_feature 1..2238: note = synthetically generated sequence
  source 1..2238: mol_type = other DNA

SEQ ID NO: 24 - protein, 745 aa, synthetic construct; identical to SEQ ID NO: 18
  REGION 1..745: note = synthetically generated sequence

SEQ ID NO: 25 - DNA, 2238 bp, synthetic construct
  misc_feature 1..2238: note = synthetically generated sequence
  source 1..2238: mol_type = other DNA
atggctgccgatggttatcttccagattggctcgaggacactctctctgaaggaataagacagtggtggaagctcaaacctggcccaccaccaccaaagcccgcagagcggcataaggacgacagcaggggtcttgtgcttcctgggtacaagtacctcggacccttcaacggactcgacaagggagagccggtcaacgaggcagacgccgcggccctcgagcacgacaaagcctacgaccggcagctcgacagcggagacaacccgtacctcaagtacaaccacgccgacgcggagtttcaggagcgccttaaagaagatacgtcttttgggggcaacctcggacgagcagtcttccaggcgaaaaagagggttcttgaacctctgggcctggttgaggaacctgttaagacggctccgggaaaaaagaggccggtagagcactctcctgtggagccagactcctcctcgggaaccggaaaggcgggccagcagcctgcaagaaaaagattgaattttggtcagactggagacgcagactcagtacctgacccccagcctctcggacagccaccagcagccccctctggtctgggagctaatacgatggctacaggcagtggcgcaccaatggcagacaataacgagggcgccgacggagtgggtaattcctcgggaaattggcattgcgattccacatggatgggcgacagagtcatcaccaccagcacccgaacctgggccctgcccacctacaacaaccacctctacaaacaaatttccagccaatcaggagcctcgaacgacaatcactactttggctacagcaccccttgggggtattttgacttcaacagattccactgccacttttcaccacgtgactggcaaagactcatcaacaacaactggggattccgacccaagagactcaacttcaagctctttaacattcaagtcaaagaggtcacgcagaatgacggtacgacgacgattgccaataaccttaccagcacggttcaggtgtttactgactcggagtaccagctcccgtacgtcctcggctcggcgcatcaaggatgcctcccgccgttcccagcagacgtcttcatggtgccacagtatggatacctcaccctgaacaacgggagtcaggcagtaggacgctcttcattttactgcctggagtactttccttctcagatgctgcgtaccggaaacagctttaccttcagctacacttttgaggacgttcctttccacagcagctacgctcacagccagagtctggaccgtctcatgaatcctctcatcgaccagtacctgtattacttgagcagaacaaacactccaagtggaaccaccacgcagtcaaggcttcagttttctcaggccggagcgagtgacattcgggaccagtctaggaactggcttcctggaccctgttaccgccagcagcgagtatcaaagacatctgcggataacaacaacagtgaatactcgtggactggagctaccaagtaccacctcaatggcagagactctctggtgaatccgggcccggccatggcaagccacaaggacgatgaagaaaagttttttcctcagagcggggttctcatctttgggaagcaaggctcagagaaaacaaatgtggacattgaaaaggtcatgattacagacgaagaggaaatcaggacaaccaatcccgtggctacggagcagtatggttctgtatctaccaacctccagagaggcaacctagcaatctccgaccagacaaaacacgctaggcaagcagctaccgcagatgtcaacacacaaggcgttcttccaggcatggtctggcaggacagagatgtgtaccttcaggggcccatctgggcaaagattccacacacggacggacattttcacccctctcccctcatgggtggattcggacttaaacaccctcctccccagattctcatcaagaacaccccggtacctgcgaatccttcgaccaccttcagtgcggcaaagtttgcttccttcatcacacagtactccacgggacaggtcagcgtggagatcgagtgggagctgcagaaggaaaacagcaaacgctggaatcccgaaattcagtacacttccaactacaacaagtctattaatgtggactttactgtggacactaatggcgtgtattcagagcctcgccccattggcaccagatacctgactcgtaatctgtaa

SEQ ID NO: 26 - protein, 745 aa, synthetic construct
  REGION 1..745: note = synthetically generated sequence
MAADGYLPDWLEDTLSEGIRQWWKLKPGPPPPKPAERHKDDSRGLVLPGYKYLGPFNGLDKGEPVNEADAAALEHDKAYDRQLDSGDNPYLKYNHADAEFQERLKEDTSFGGNLGRAVFQAKKRVLEPLGLVEEPVKTAPGKKRPVEHSPVEPDSSSGTGKAGQQPARKRLNFGQTGDADSVPDPQPLGQPPAAPSGLGANTMATGSGAPMADNNEGADGVGNSSGNWHCDSTWMGDRVITTSTRTWALPTYNNHLYKQISSQSGASNDNHYFGYSTPWGYFDFNRFHCHFSPRDWQRLINNNWGFRPKRLNFKLFNIQVKEVTQNDGTTTIANNLTSTVQVFTDSEYQLPYVLGSAHQGCLPPFPADVFMVPQYGYLTLNNGSQAVGRSSFYCLEYFPSQMLRTGNSFTFSYTFEDVPFHSSYAHSQSLDRLMNPLIDQYLYYLSRTNTPSGTTTQSRLQFSQAGASDIRDQSRNWLPGPCYRQQRVSKTSADNNNSEYSWTGATKYHLNGRDSLVNPGPAMASHKDDEEKFFPQSGVLIFGKQGSEKTNVDIEKVMITDEEEIRTTNPVATEQYGSVSTNLQRGNLAISDQTKHARQAATADVNTQGVLPGMVWQDRDVYLQGPIWAKIPHTDGHFHPSPLMGGFGLKHPPPQILIKNTPVPANPSTTFSAAKFASFITQYSTGQVSVEIEWELQKENSKRWNPEIQYTSNYNKSINVDFTVDTNGVYSEPRPIGTRYLTRNL

SEQ ID NO: 27 - DNA, 2238 bp, synthetic construct
  misc_feature 1..2238: note = synthetically generated sequence
  source 1..2238: mol_type = other DNA
atggctgccgatggttatcttccagattggctcgaggacactctctctgaaggaataagacagtggtggaagctcaaacctggcccaccaccaccaaagcccgcagggcggcataaggacgacagcaggggtcttgtgcttcctgggtacaagtacctcggacccttcaacggactcgacaagggagagccggtcaacgaggcagacgccgcggccctcgagcacgacaaagcctacgaccggcagctcgacagcggagacaacccgtacctcaagtacaaccacgccgacgcggagtttcaggagcgccttaaagaagatacgtcttttgggggcaacctcggacgagcagtcttccaggcgaaaaagagggttcttgaacctctgggcctggttgaggaacctgttaagacggctccgggaaaaaagaggccggtagagcactctcctgtggagccagactcctcctcgggaaccggaaaggcgggccagcagcctgcaagaaaaagattgaattttggtcagactggagacgcagactcagaacctgacccccagcctctcggacagccaccagcagccccctctggtctgggaactaatacgatggctacaggcagtggcgcaccaatggcagacaataacgagggcgccgacggagtgggtaattcctcgggaaattggcattgcgattccacatggatgggcgacagagtcatcaccaccagcacccgaacctgggccctgcccacctacaacaaccacctctacaaacaaatttccagccaatcaggagcctcgaacgacaatcactactttggctacagcaccccttgggggtattttgacttcaacagattccactgccacttttcaccacgtgactggcaaagactcatcaacaacaactggggattccgacccaagagactcaacttcaagctctttaacattcaagtcaaagaggtcacgcagaatgacggtacgacgacgattgccaataaccttaccagcacggttcaggtgtttactgactcggagtaccagctcccgtacgtcctcggctcggcgcatcaaggatgcctcccgccgttcccagcagacgtcttcatggtgccacagtatggatacctcaccctgaacaacgggagtcaggcagtaggacgctcttcattttactgcctggagtactttccttctcagatgctgcgtaccggaaacaactttaccttcagctacacttttgaggacgttcctttccacagcagctacgctcacagccagagtctggaccgtctcatgaatcctctcatcgaccagtacctgtattacttgagcagaacaaacactccaagtggaaccaccacgcagtcaaggcttcagttttctcaggccggagcgagtgacattcgggaccagtctaggaactggcttcctggaccctgttaccgccagcagcgagtatcaaagacacctgcggataacaacaacagtgaatactcgtggactggagctaccaagtaccacctcaatggcagagactctctggtgaatccgggcccggccatggcaagccacaaggacgatgaagaaaagttttttcctcagagcggggttctcatctttgggaagcaaggctcagagaaaacaaatgtggacattgaaaaggtcatgattacagacgaagaggaaatcaggacaaccaatcccgtggctacggagcagtatggttctgtatctaccaacctccagagaggcaacctagcaaaccaagactacacaaaaactgctaggcaagcagctaccgcagatgtcaacacacaaggcgttcttccaggcatggtctggcaggacagagatgtgtaccttcaggggcccatctgggcaaagattccacacacggacggacattttcacccctctcccctcatgggtggattcggacttaaacaccctcctccccagattctcatcaagaacaccccggtacctgcgaatccttcgaccaccttcagtgcggcaaagtttgcttccttcatcacacagtactccacgggacaggtcagcgtggagatcgagtgggagctgcagaaggaaaacagcaaacgctggaatcccgaaattcagtacacttccaactacaacaagtctattaatgtggactttactgtggacactaatggcgtgtattcagagcctcgccccattggcaccagatacctgactcgtaatctgtaa

SEQ ID NO: 28 - protein, 745 aa, synthetic construct
  REGION 1..745: note = synthetically generated sequence
MAADGYLPDWLEDTLSEGIRQWWKLKPGPPPPKPAGRHKDDSRGLVLPGYKYLGPFNGLDKGEPVNEADAAALEHDKAYDRQLDSGDNPYLKYNHADAEFQERLKEDTSFGGNLGRAVFQAKKRVLEPLGLVEEPVKTAPGKKRPVEHSPVEPDSSSGTGKAGQQPARKRLNFGQTGDADSEPDPQPLGQPPAAPSGLGTNTMATGSGAPMADNNEGADGVGNSSGNWHCDSTWMGDRVITTSTRTWALPTYNNHLYKQISSQSGASNDNHYFGYSTPWGYFDFNRFHCHFSPRDWQRLINNNWGFRPKRLNFKLFNIQVKEVTQNDGTTTIANNLTSTVQVFTDSEYQLPYVLGSAHQGCLPPFPADVFMVPQYGYLTLNNGSQAVGRSSFYCLEYFPSQMLRTGNNFTFSYTFEDVPFHSSYAHSQSLDRLMNPLIDQYLYYLSRTNTPSGTTTQSRLQFSQAGASDIRDQSRNWLPGPCYRQQRVSKTPADNNNSEYSWTGATKYHLNGRDSLVNPGPAMASHKDDEEKFFPQSGVLIFGKQGSEKTNVDIEKVMITDEEEIRTTNPVATEQYGSVSTNLQRGNLANQDYTKTARQAATADVNTQGVLPGMVWQDRDVYLQGPIWAKIPHTDGHFHPSPLMGGFGLKHPPPQILIKNTPVPANPSTTFSAAKFASFITQYSTGQVSVEIEWELQKENSKRWNPEIQYTSNYNKSINVDFTVDTNGVYSEPRPIGTRYLTRNL

SEQ ID NO: 29 - DNA, 2238 bp, synthetic construct
  misc_feature 1..2238: note = synthetically generated sequence
  source 1..2238: mol_type = other DNA
atggctgccgatggttatcttccagattggctcgaggacactctctctgaaggaataagacagtggtggaagctcaaacctggcccaccaccaccaaagcccgcagagcggcataaggacgacagcaggggtcttgtgcttcctgggtacaagtacctcggacccttcaacggactcgacaagggagagccggtcaacgaggcagacgccgcggccctcgagcacgacaaagcctacgaccggcagctcgacagcggagacaacccgtacctcaagtacaaccacgccgacgcggagtttcaggagcgccttaaagaagatacgtcttttgggggcaacctcggacgagcagtcttccaggcgaaaaagagggttcttgaacctctgggcctggttgaggaacctgttaagacggctccgggaaaaaagaggccggtagagcactctcctgtggagccagactcctcctcgggaaccggaaaggcgggccagcagcctgcaagaaaaagattgaattttggtcagactggagacgcagactcagtacctgaccccaggcctctcggacagccaccagcagccccctctggtctgggaactaatacgatggctacaggcagtggcgcaccaatggcagacaataacgagggcgccgacggagtgggtaattcctcgggaaattggcattgcgattccacatggatgggcgacagagtcatcaccaccagcacccgaacctgggccctgcccacctacaacaaccacctctacaaacaaatttccagccaatcaggagcctcgaacgacaatcactactttggctacagcaccccttgggggtattttgacttcaacagattccactgccacttttcaccacgtgactggcaaagactcatcaacaacaactggggattccgacccaagagactcaacttcaagctctttaacattcaagtcaaagaggtcacgcagaatgacggtacgacgacgattgccaataaccttaccagcacggttcaggtgtttactgactcggagtaccagctcccgtacgtcctcggctcggcgcatcaaggatgcctcccgccgttcccagcagacgtcttcatggtgccacagtatggatacctcaccctgaacgacgggagtcaggcagtaggacgctcttcattttactgcctggagtactttccttctcagatgctgcgtaccggaaacaactttaccttcagctacacttttgaggacgttcctttccacagcagctacgctcacagccagagtctggaccgtctcatgaatcctctcatcgaccagtacctgtattacttgagcagaacaaacactccaagtggaaccaccacgcagtcaaggcttcagttttctcaggccggagcgagtgacattcgggaccagtctaggaactggcttcctggaccctgttaccgccagcagcgagtatcaaagacatctgcggataacaacaacagtgaatactcgtggactggagctaccaagtaccacctcaatggcagagactctctggtgaatccgggcccggccatggcaagccacaaggacgatgaagaaaagttttttcctcagagcggggttctcatctttgggaagcaaggctcagagaaaacaaatgtggacattgaaaaggtcatgattacagacgaagaggaaatcaggacaaccaatcccgtggctacggagcagtatggttctgtatctaccaacctccagagaggcaacctagcaatctccgaccagacaaaacacgctaggcaagcagctaccgcaaatgtcaacacacaaggcgttcttccaggcatggtctggcaggacagagatgtgtaccttcaggggcccatctgggcaaagattccacacacggacggacattttcacccctctcccctcatgggtggattcggacttaaacaccctcctccccagattctcatcaagaacaccccggtacctgcgaatccttcgaccaccttcagtgcggcaaagtttgcttccttcatcacacagtactccacgggacaggtcagcgtggagatcgagtgggagctgcagaaggaaaacagcaaacgctggaatcccgaaattcagtacacttccaactacaacaagtctattaatgtggactttactgtggacactaatggcgtgtattcagagcctcgccccattggcaccagatacctgactcgtaatctgtaa

SEQ ID NO: 30 - protein, 745 aa, synthetic construct
  REGION 1..745: note = synthetically generated sequence
MAADGYLPDWLEDTLSEGIRQWWKLKPGPPPPKPAERHKDDSRGLVLPGYKYLGPFNGLDKGEPVNEADAAALEHDKAYDRQLDSGDNPYLKYNHADAEFQERLKEDTSFGGNLGRAVFQAKKRVLEPLGLVEEPVKTAPGKKRPVEHSPVEPDSSSGTGKAGQQPARKRLNFGQTGDADSVPDPRPLGQPPAAPSGLGTNTMATGSGAPMADNNEGADGVGNSSGNWHCDSTWMGDRVITTSTRTWALPTYNNHLYKQISSQSGASNDNHYFGYSTPWGYFDFNRFHCHFSPRDWQRLINNNWGFRPKRLNFKLFNIQVKEVTQNDGTTTIANNLTSTVQVFTDSEYQLPYVLGSAHQGCLPPFPADVFMVPQYGYLTLNDGSQAVGRSSFYCLEYFPSQMLRTGNNFTFSYTFEDVPFHSSYAHSQSLDRLMNPLIDQYLYYLSRTNTPSGTTTQSRLQFSQAGASDIRDQSRNWLPGPCYRQQRVSKTSADNNNSEYSWTGATKYHLNGRDSLVNPGPAMASHKDDEEKFFPQSGVLIFGKQGSEKTNVDIEKVMITDEEEIRTTNPVATEQYGSVSTNLQRGNLAISDQTKHARQAATANVNTQGVLPGMVWQDRDVYLQGPIWAKIPHTDGHFHPSPLMGGFGLKHPPPQILIKNTPVPANPSTTFSAAKFASFITQYSTGQVSVEIEWELQKENSKRWNPEIQYTSNYNKSINVDFTVDTNGVYSEPRPIGTRYLTRNL

SEQ ID NO: 31 - DNA, 2188 bp, synthetic construct
  misc_feature 1..2188: note = synthetically generated sequence
  source 1..2188: mol_type = other DNA
atggctgccgatggttatcttccagattggctcgaggacactctctctgaaggaataagacagtggtggaagctcaaacctggcccaccaccaccaaagcccgcagagcggcataaggacgacagcaggggtcttgtgcttcctgggtacaagtacctcggacccttcaacggactcgacaagggagagccggtcaacgaggcagacgccgcggccctcgagcacgacaaagcctacgaccggcagctcgacagcggagacaacccgtacctcaagtacaaccacgccgacgcggagtttcaggagcgccttaaagaagatacgtcttttgggggcaacctcggacgagcagtcttccaggcgaaaaagagggttcttgaacctctgggcctggttgaggaacctgttaagacggctccgggaaaaaagaggccggtagagcactctcctgtggagccagactcctcctcgggaaccggaaaggcgggccagcagcctgcaagaaaaagattgaattttggtcagactggagacgcagactcagtacctgacccccagcctctcggacagccaccagcagccccctctggtctgggaactaatacgatggctacaggcagtggcgcaccaatggcagacaataacgagggcgccgacggagtgggtaattcctcgggaaattggcattgcgattccacatggctgggcgacagagtcatcaccaccagcacccgaacctgggccctgcccacctacaacaaccacctctacaaacaaatttccagccaatcaggagcctcgaacgacaatcactactttggctacagcaccccttgggggtattttgactacaacagattccactgccacttttcaccacgtgactggcaaagactcatcaacaacaactggggattccgacccaagagactcaacttcaagctctttaacattcaagtcaaagaggtcacgcagaatgacggtacgacgacgattgccaataaccttaccagcacggttcaggtgtttactgactcggagtaccagctcccgtacgtcctcggctcggcgcatcaaggatgcctcccgccgttcccagcagacgtcttcatggtgccacagtatggatacctcaccctgaacaacgggagtcaggcagtaggacgctcttcattttactgcctggagtactttccttctcagatgctgcgtaccggaaacaactttaccttcagctacacttttgaggacgttcctttccacagcagctacgctcacagccagagtctggaccgtctcatgaatcctctcatcgaccagtacctgtattacttgagcagaacaaacactccaagtggaaccaccacgcagtcaaggcttcagttttctcaggccggagcgagtgacattcgggaccagtctaggaactggcttcctggaccctgttaccgccagcagcgagtatcaaagacatctgcggataacaacaacagtgaatactcgtggactggagctaccaagtaccacctcaatggcagagactctctggtgaatccgggcccggccatggcaagccacaaggacgatgaagaaaagttttttcctcagagcggggttctcatctttgggaagcaaggctcagagaaaacaaatgtggacattgaaaaggtcatgattacagacgaagaggaaatcaggacaaccaatcccgtggctacggagcagtatggttctgtatctaccaacctccagagaggcaacctagcagaccaagactacacaaaaactgctaggcaagcaggacagagatgtgtaccttcaggggcccatctgggcaaagattccacacacggacggacattttcacccctctcccctcatgggtggattcggacttaaacaccctcctccccagattctcatcaagaacaccccggtacctgcgaatccttcgaccaccttcagtgcggcaaagtttgcttccttcatcacacagtactccacgggacaggtcagcgtggagatcgagtgggagctgcagaaggaaaacagcaaacgctggaatcccgaaattcagtacacttccaactacaacaagtctattaatgtggactttactgtggacactaatggcgtgtattcagagcctcgccccattggcaccagatacctgactcgtaatctgtaa

SEQ ID NO: 32 - protein, 745 aa, synthetic construct
  REGION 1..745: note = synthetically generated sequence
MAADGYLPDWLEDTLSEGIRQWWKLKPGPPPPKPAERHKDDSRGLVLPGYKYLGPFNGLDKGEPVNEADAAALEHDKAYDRQLDSGDNPYLKYNHADAEFQERLKEDTSFGGNLGRAVFQAKKRVLEPLGLVEEPVKTAPGKKRPVEHSPVEPDSSSGTGKAGQQPARKRLNFGQTGDADSVPDPQPLGQPPAAPSGLGTNTMATGSGAPMADNNEGADGVGNSSGNWHCDSTWLGDRVITTSTRTWALPTYNNHLYKQISSQSGASNDNHYFGYSTPWGYFDYNRFHCHFSPRDWQRLINNNWGFRPKRLNFKLFNIQVKEVTQNDGTTTIANNLTSTVQVFTDSEYQLPYVLGSAHQGCLPPFPADVFMVPQYGYLTLNNGSQAVGRSSFYCLEYFPSQMLRTGNNFTFSYTFEDVPFHSSYAHSQSLDRLMNPLIDQYLYYLSRTNTPSGTTTQSRLQFSQAGASDIRDQSRNWLPGPCYRQQRVSKTSADNNNSEYSWTGATKYHLNGRDSLVNPGPAMASHKDDEEKFFPQSGVLIFGKQGSEKTNVDIEKVMITDEEEIRTTNPVATEQYGSVSTNLQRGNLADQDYTKTARQAATADVNTQGVLPGMVWQDRDVYLQGPIWAKIPHTDGHFHPSPLMGGFGLKHPPPQILIKNTPVPANPSTTFSAAKFASFITQYSTGQVSVEIEWELQKENSKRWNPEIQYTSNYNKSINVDFTVDTNGVYSEPRPIGTRYLTRNL

SEQ ID NO: 33 - DNA, 2238 bp, synthetic construct
  misc_feature 1..2238: note = synthetically generated sequence
  source 1..2238: mol_type = other DNA
atggctgccgatggttatcttccagattggctcgaggacactctctctgaaggaataagacagtggtggaagctcaaacctggcccaccaccaccaaagcccgcagagcggcataaggacgacagcaggggtcttgtgcttcctgggtacaagtacctcggacccttcaacggactcgacaagggagagccggtcaacgaggcagaggccgcggccctcgagcacgacaaagcctacgaccggcagctcgacagcggagacaacccgtacctcaagtacaaccacgccgacgcggagtttcaggagcgccttaaagaagatacgtcttttgggggcaacctcggacgagcagtcttccaggcgaaaaagagggttcttgaacctctgggcctggttgaggaacctgttaagacggctccgggaaaaaagaggccggtagagcactctcctgtggagccagactcctcctcgggaaccggaaaggcgggccagcagcctgcaagaaaaagattgaattttggtcagactggagacgcagactcagaacctgacccccagcctctcggacagccaccagcagccccctctggtctgggaactaatacgatggctacaggcagtggcgcaccaatggcagacaataacgagggcgccgacggagtgggtaattcctcgggaaattggcattgcgattccacatggatgggcgacagagtcatcaccaccagcacccgaacctgggccctgcccacctacaacaaccacctctacaaacaaatttccagccaatcaggagcctcgaacgacaatcactactttggctacagcaccccttgggggtattttgacttcaacagattccactgccacttttcaccacgtgactggcaaagactcatcaacaacaactggggattccgacccaagagactcaacttcaagctctttaacattcaagtcaaagaggtcacgcagaatgacggtacgacgacgattgccaataaccttaccagcacggttcaggtgtttactgactcggagtaccagctcccgtacgtcctcggctcggcgcatcaaggatgcctcccgccgttcccagcagacgtcttcatggtgccacagtatggatacctcaccctgaacaacgggagtcaggcagtaggacgctcttcattttactgcctggagtactttccttctcagatgctgcgtaccggaaacagctttaccttcagctacacttttgaggacgttcctttccacagcagctacgctcacagccagagtctggaccgtctcatgaatcctctcatcgaccagtacctgtattacttgagcagaacaaacactccaagtggaaccaccacgcagtcaaggcttcagttttctcaggccggagcgagtgacattcgggaccagtctaggaactggcttcctggaccctgttaccgccagcagcgagtatcaaagacatctgcggataacaacaacagtgaatactcgtggactggagctaccaagtaccacctcaatggcagagactctctggtgaatccgggcccggccatggcaagccacaaggacgatgaagaaaagttttttcctcagagcggggttctcatctttgggaagcaaggctcagagaaaacaaatgtggacattgaaaaggtcatgattacagacgaagaggaaatcaggacaaccaatcccgtggctacggagcagtatggttctgtatctaccaacctccagagaggcaacctagcaatctccgaccagacaaaacacgctaggcaagcagctaccgcagatgtcaacacacaaggcgttcttccaggcatggtctggcaggacagagatgtgtaccttcaggggcccatctgggcaaagattccacacacggacggacattttcacccctctcccctcatgggtggattcggacttaaacaccctcctccccagattctcatcaagaacaccccggtacctgcgaatccttcgaccaccttcagtgcggcaaagtttgcttccttcatcacacagtactccacgggacaggtcagcgtggagatcgagtgggagctgcagaaggaaaacagcaaacgctggaatcccgaaattcagtacacttccaactacaacaagtctattaatgtggactttactgtggacactaatggcgtgtattcagagcctcgccccattggcaccagatacctgactcgtaatctgtaa

SEQ ID NO: 34 - protein, 745 aa, synthetic construct
  REGION 1..745: note = synthetically generated sequence
MAADGYLPDWLEDTLSEGIRQWWKLKPGPPPPKPAERHKDDSRGLVLPGYKYLGPFNGLDKGEPVNEAEAAALEHDKAYDRQLDSGDNPYLKYNHADAEFQERLKEDTSFGGNLGRAVFQAKKRVLEPLGLVEEPVKTAPGKKRPVEHSPVEPDSSSGTGKAGQQPARKRLNFGQTGDADSEPDPQPLGQPPAAPSGLGTNTMATGSGAPMADNNEGADGVGNSSGNWHCDSTWMGDRVITTSTRTWALPTYNNHLYKQISSQSGASNDNHYFGYSTPWGYFDFNRFHCHFSPRDWQRLINNNWGFRPKRLNFKLFNIQVKEVTQNDGTTTIANNLTSTVQVFTDSEYQLPYVLGSAHQGCLPPFPADVFMVPQYGYLTLNNGSQAVGRSSFYCLEYFPSQMLRTGNSFTFSYTFEDVPFHSSYAHSQSLDRLMNPLIDQYLYYLSRTNTPSGTTTQSRLQFSQAGASDIRDQSRNWLPGPCYRQQRVSKTSADNNNSEYSWTGATKYHLNGRDSLVNPGPAMASHKDDEEKFFPQSGVLIFGKQGSEKTNVDIEKVMITDEEEIRTTNPVATEQYGSVSTNLQRGNLAISDQTKHARQAATADVNTQGVLPGMVWQDRDVYLQGPIWAKIPHTDGHFHPSPLMGGFGLKHPPPQILIKNTPVPANPSTTFSAAKFASFITQYSTGQVSVEIEWELQKENSKRWNPEIQYTSNYNKSINVDFTVDTNGVYSEPRPIGTRYLTRNL

SEQ ID NO: 35 - DNA, 2238 bp, synthetic construct
  misc_feature 1..2238: note = synthetically generated sequence
  source 1..2238: mol_type = other DNA
atggctgccgatggttatcttccagattggctcgaggacactctctctgaaggaataagacagtggtggaagctcaaacctggcccaccaccaccaaagcccgcagagcggcataaggacgacagcaggggtcttgtgcttcctgggtacaagtacctcggacccttcaacggactcgacaagggagagccggtcaacgaggcagacgccgcggccctcgagcacgacaaagcctacgaccggcagctcgacagcggagacaacccgtacctcaagtacaaccacgccgacgcggagtttcaggagcgccttaaagaagatacgtcttttgggggcaacctcggacgagcagtcttccaggcgaaaaagagggttcttgaacctctgggcctggttgaggaacctgttaagacggctccgggaaaaaagaggccggtagagcactctcctgtggagccagactcctcctcgggaaccggaaaggcgggccagcagcctgcaagaaaaagattgaattttggtcagactggagacgcagactcagaacctgacccccagcctctcggacagccaccagcagccccctctggtctgggaactaatacgatggctacaggcagtggcgcaccaatggcagacaataacgagggcgccgacggagtgggtaattcctcgggaaattggcattgcgattccacatggatgggcgacagagtcatcaccaccagcacccgaacctgggccctgcccacctacaacaaccacctctacaaacaaatttccagccaatcaggagcctcgaacgacaatcactactttggctacagcaccccttgggggtattttgacttcaacagattccactgccacttttcaccacgtgactggcaaagactcatcaacaacaactggggattccgacccaagagactcaacttcaagctctttaacattcaagtcaaagaggtcacgcagaatgacggtacgacgacgattgccaataaccttaccagcacggttcaggtgtttactgactcggagtaccagctcccgtacgtcctcggctcggcgcatcaaggatgcctcccgccgttcccagcagacgtcttcatggtgccacagtatggatacctcaccctgaacaacgggagtcaggcagtaggacgctcttcattttactgcctggagtactttccttctcagatgctgcgtaccggaaacaactttaccttcagctacacttttgaggacgttcctttccacagcagctacgctcacagccagagtctggaccgtctcatgaatcctctcatcgaccagtacctgtattacttgagcagaacaaacactccaagtggaaccaccacgcagtcaaggcttcagttttctcaggccggagcgagtgacattcgggaccagtctaggaactggcttcctggaccctgttaccgccagcagcgagtatcaaagacatctgcggataactacaacagtgaatactcgtggactggagctaccaagtaccacctcaatggcagagactctctggtgaatccgggcccggccatggcaagccacaaggacgatgaagaaaagttttttcctcagagcggggttctcatctttgggaagcaaggctcagagaaaacaaatgtggacattgaaaaggtcatgattacagacgaagaggaaatcaggacaaccaatcccgtggctacggagcagtatggttctgtatctaccaacctccagagaggcaacctagcaatctccgaccagacaaaacacgctaggcaagcagctaccgcagatgtcaacacacaaggcgttcttccaggcatggtctggcaggacagagatgtgtaccttcaggggcccatctgggcaaagattccacacacggacggacattttcacccctctcccctcatgggtggattcggacttaaacaccctcctccccagattctcatcaagaacaccccggtacctgcgaatccttcgaccaccttcagtgcggcaaagtttgcttccttcatcacacagtactccacgggacaggtcagcgtggagatcgagtgggagctgcagaaggaaaacagcaaacgctggaatcccgaaattcagtacacttccaactacaacaagtctattaatgtggactttactgtggacactaatggcgtgtattcagagcctcgccccattggcaccagatacctgactcgtaatctgtaa

SEQ ID NO: 36 - protein, 745 aa, synthetic construct
  REGION 1..745: note = synthetically generated sequence
MAADGYLPDWLEDTLSEGIRQWWKLKPGPPPPKPAERHKDDSRGLVLPGYKYLGPFNGLDKGEPVNEADAAALEHDKAYDRQLDSGDNPYLKYNHADAEFQERLKEDTSFGGNLGRAVFQAKKRVLEPLGLVEEPVKTAPGKKRPVEHSPVEPDSSSGTGKAGQQPARKRLNFGQTGDADSEPDPQPLGQPPAAPSGLGTNTMATGSGAPMADNNEGADGVGNSSGNWHCDSTWMGDRVITTSTRTWALPTYNNHLYKQISSQSGASNDNHYFGYSTPWGYFDFNRFHCHFSPRDWQRLINNNWGFRPKRLNFKLFNIQVKEVTQNDGTTTIANNLTSTVQVFTDSEYQLPYVLGSAHQGCLPPFPADVFMVPQYGYLTLNNGSQAVGRSSFYCLEYFPSQMLRTGNNFTFSYTFEDVPFHSSYAHSQSLDRLMNPLIDQYLYYLSRTNTPSGTTTQSRLQFSQAGASDIRDQSRNWLPGPCYRQQRVSKTSADNYNSEYSWTGATKYHLNGRDSLVNPGPAMASHKDDEEKFFPQSGVLIFGKQGSEKTNVDIEKVMITDEEEIRTTNPVATEQYGSVSTNLQRGNLAISDQTKHARQAATADVNTQGVLPGMVWQDRDVYLQGPIWAKIPHTDGHFHPSPLMGGFGLKHPPPQILIKNTPVPANPSTTFSAAKFASFITQYSTGQVSVEIEWELQKENSKRWNPEIQYTSNYNKSINVDFTVDTNGVYSEPRPIGTRYLTRNL

SEQ ID NO: 37 - DNA, 2238 bp, synthetic construct
  misc_feature 1..2238: note = synthetically generated sequence
  source 1..2238: mol_type = other DNA
atggctgccgatggttatcttccagattggctcgaggacactctctctgaaggaataagacagtggtggaagctcaaacctggcccaccaccaccaaagcccgcagagcggcataaggacgacagcaggggtcttgtgcttcctgggtacaagtacctcggacccttcaacggactcgacaagggagagccggtcaacgccgcagacgccgcggccctcgagcacgacaaagcctacgaccggcagctcgacagcggagacaacccgtacctcaagtacaaccacgccgacgcggagtttcaggagcgccttaaagaagatacgtcttttgggggcaacctcggacgagcagccttccaggcgaaaaagagggttcttgaacctctgggcctggttgaggaacctgttaagacggctccgggaaaaaagaggccggtagagcactctcctgtggagccagactcctcctcgggaaccggaaaggcgggccagcagcctgcaagaaaaagattgaattttggtcagactggagacgcagactcaatacctgacccccagcctctcggacagccaccagcagccccctctggtctgggaactaatacgatggctacaggcagtggcgcaccaatggcagacaataacgagggcgccgacggagtgggtaattcctcgggaaattggcattgcgattccacatggatgggcgacagagtcatcaccaccagcacccgaacctgggccctgcccacctacaacaaccacctctacaaacaaatttccagccaatcaggagcctcgaacgacaatcactactttggctacagcaccccttgggggtattttgacttcaacagattccactgccacttttcaccacgtgactggcaaagactcatcaacaacaactggggattccgacccaagagactcaacttcaagctctttaacattcaagtcaaagaggtcacgcagaatgacggtacgacgacgattgccaataaccttaccagcacggttcaggtgtttactgactcggagtaccagctcccgtacgtcctcggctcggcgcatcaaggatgcctcccgccgttcccagcagacgtcttcatggtgccacagtatggatacctcaccctgaacaacgggagtcaggcagtaggacgctcttcattttactgcctggagtactttccttctcagatgctgcgtaccggaaacaactttaccttcagctacacttttgaggacgttcctttccacagcagctacgctcacagccagagtctggaccgtctcatgaatcctctcatcgaccagtacctgtattacttgagcagaacaaacactccaagtggaaccaccacgcagtcaaggcttcagttttctcaggccggagcgagtgacattcgggaccagtctaggaactggcttcctggaccctgttaccgccagcagcgagtatcaaagacatctgcggataacaacaacagtgaatactcgtggactggagctaccaagtaccacctcaatggcagagactctctggtgaatccgggcccggccatggcaagccacaaggacgatgaagaaaagttttttcctcagagcggggttctcatctttgggaagcaaggctcagagaaaacaaatgtggacattgaaaaggtcatgattacagacgaagaggaaatcaggacaaccaatcccgtggctacggagcagtatggttctgtatctaccaacctccagagaggcaacctagcacagcctgacgccacaaaaaacgctaggcaagcagctaccgcagatgtcaacacacaaggcgttcttccaggcatggtctggcaggacagagatgtgtaccttcaggggcccatctgggcaaagattccacacacggacggacattttcacccctctcccctcatgggtggattcggacttaaacaccctcctccccagattctcatcaagaacaccccggtacctgcgaatccttcgaccaccttcagtgcggcaaagtttgcttccttcatcacacagtactccacgggacaggtcagcgtggagatcgagtgggagctgcagaaggaaaacagcaaacgctggaatcccgaaattcagtacacttccaactacaacaagtctattaatgtggactttactgtggacactaatggcgtgtattcagagcctcgccccattggcaccagatacctgactcgtaatctgtaa

SEQ ID NO: 38 - protein, 745 aa, synthetic construct
  REGION 1..745: note = synthetically generated sequence
MAADGYLPDWLEDTLSEGIRQWWKLKPGPPPPKPAERHKDDSRGLVLPGYKYLGPFNGLDKGEPVNAADAAALEHDKAYDRQLDSGDNPYLKYNHADAEFQERLKEDTSFGGNLGRAAFQAKKRVLEPLGLVEEPVKTAPGKKRPVEHSPVEPDSSSGTGKAGQQPARKRLNFGQTGDADSIPDPQPLGQPPAAPSGLGTNTMATGSGAPMADNNEGADGVGNSSGNWHCDSTWMGDRVITTSTRTWALPTYNNHLYKQISSQSGASNDNHYFGYSTPWGYFDFNRFHCHFSPRDWQRLINNNWGFRPKRLNFKLFNIQVKEVTQNDGTTTIANNLTSTVQVFTDSEYQLPYVLGSAHQGCLPPFPADVFMVPQYGYLTLNNGSQAVGRSSFYCLEYFPSQMLRTGNNFTFSYTFEDVPFHSSYAHSQSLDRLMNPLIDQYLYYLSRTNTPSGTTTQSRLQFSQAGASDIRDQSRNWLPGPCYRQQRVSKTSADNNNSEYSWTGATKYHLNGRDSLVNPGPAMASHKDDEEKFFPQSGVLIFGKQGSEKTNVDIEKVMITDEEEIRTTNPVATEQYGSVSTNLQRGNLAQPDATKNARQAATADVNTQGVLPGMVWQDRDVYLQGPIWAKIPHTDGHFHPSPLMGGFGLKHPPPQILIKNTPVPANPSTTFSAAKFASFITQYSTGQVSVEIEWELQKENSKRWNPEIQYTSNYNKSINVDFTVDTNGVYSEPRPIGTRYLTRNL

SEQ ID NO: 39 - DNA, 2238 bp, synthetic construct
  misc_feature 1..2238: note = synthetically generated sequence
  source 1..2238: mol_type = other DNA
atggctgccgatggttatcttccagattggctcgtggacactctctctgaaggaataagacagtggtggaagctcaaacctggcccaccaccaccaaagcccgcagagcggcataaggacgacagcaggggtcttgtgcttcctgggtacaagtacctcggacccttcaacggactcgacaagggagagccggtcaacgccgcagacgccgcggccctcgagcacgacaaagcctacgaccggcagctcgacagcggagacaacccgtacctcaagtacaaccacgccgacgcggagtttcaggagcgccttaaagaagatacgtcttttgggggcaacctcggacgagcagtcttccaggcgaaaaagagggttcttgaacctctgggcctggttgaggaacctgttgagacggctccgggaaaaaagaggccggtagagcactctcctgtggagccagactcctcctcgggaaccggaaaggcgggccagcagcctgcaagaaaaagattgaattttggtcagactggagacgcagactcagtacctgacccccagcctctcggacagccaccagcagccccctctggtctgggaactaatacgatggctacaggcggtggcgcaccaatggcagacaataacgagggcgccgacggagtgggtaattcctcgggaaattggcattgcgattccacatggatgggcgacagagtcatcaccaccagcacccgaacctgggccctgcccacctacaacaaccacctctacaaacaaatttccagccaatcaggagcctcgaacgacaatcactactttggctacagcaccccttgggggtattttgacttcaacagattccactgccacttttcaccacgtgactggcaaagactcatcaacaacaactggggattccgacccaagagactcaacttcaagctctttaacattcaagtcaaagaggtcacgcagaatgacggtacgacgacgattgccaataaccttaccagcacggttcaggtgtttactgactcggagtaccagctcccgtacgtcctcggctcggcgcatcaaggatgcctcccgccgttcccagcagacgtcttcatggtgccacagtatggatacctcaccctgaacaacgggagtcaggcagtaggacgctcttcattttactgcctggagtactttccttctcagatgctgcgtaccggaaacaactttaccttcagctacacttttgaggacgttcctttccacagcagctacgctcacagccagagtctggaccgtctcatgaatcctctcatcgaccagtacctgtattacttgagcagaacaaacactccaagtggaaccaccacgcagtcaaggcttcagttttctcaggccggagcgagtgacattcgggaccagtctaggaactggcttcctggaccctgttaccgccagcagcgagtatcaaagacatctgcggataacaacaacagtgaatactcgtggactggagctaccaagtaccacctcaatggcagagactctctggtgaatccgggcccggccatggcaagccacaaggacgatgaagaaaagttttttcctcagagcggggttctcatctttgggaagcaaggctcagagaaaacaaatgtggacattgaaaaggtcatgattacagacgaagaggaaatcaggacaaccaatcccgtggctacggagcagtatggttctgtatctaccaacctccagagaggcaacctagcacacgacatcaccaagaatattgctaggcaagcagctaccgcagatgtcaacacacaaggcgttcttccaggcatggtctggcaggacagagatgtgtaccttcaggggcccatctgggcaaagattccacacacggacggacattttcacccctctcccctcatgggtggattcggacttaaacaccctcctccccagattctcatcaagaacaccccggtacctgcgaatccttcgaccaccttcagtgcggcaaagtttgcttccttcatcacacagtactccacgggacaggtcagcgtggagatcgagtgggagctgcagaaggaaaacagcaaacgctggaatcccgaaattcagtacacttccaactacaacaagtctattaatgtggactttactgtggacactaatggcgtgtattcagagcctcgccccattggcaccagatacctgactcgtaatctgtaa

SEQ ID NO: 40 - protein, 745 aa, synthetic construct
  REGION 1..745: note = synthetically generated sequence
MAADGYLPDWLVDTLSEGIRQWWKLKPGPPPPKPAERHKDDSRGLVLPGYKYLGPFNGLDKGEPVNAADAAALEHDKAYDRQLDSGDNPYLKYNHADAEFQERLKEDTSFGGNLGRAVFQAKKRVLEPLGLVEEPVETAPGKKRPVEHSPVEPDSSSGTGKAGQQPARKRLNFGQTGDADSVPDPQPLGQPPAAPSGLGTNTMATGGGAPMADNNEGADGVGNSSGNWHCDSTWMGDRVITTSTRTWALPTYNNHLYKQISSQSGASNDNHYFGYSTPWGYFDFNRFHCHFSPRDWQRLINNNWGFRPKRLNFKLFNIQVKEVTQNDGTTTIANNLTSTVQVFTDSEYQLPYVLGSAHQGCLPPFPADVFMVPQYGYLTLNNGSQAVGRSSFYCLEYFPSQMLRTGNNFTFSYTFEDVPFHSSYAHSQSLDRLMNPLIDQYLYYLSRTNTPSGTTTQSRLQFSQAGASDIRDQSRNWLPGPCYRQQRVSKTSADNNNSEYSWTGATKYHLNGRDSLVNPGPAMASHKDDEEKFFPQSGVLIFGKQGSEKTNVDIEKVMITDEEEIRTTNPVATEQYGSVSTNLQRGNLAHDITKNIARQAATADVNTQGVLPGMVWQDRDVYLQGPIWAKIPHTDGHFHPSPLMGGFGLKHPPPQILIKNTPVPANPSTTFSAAKFASFITQYSTGQVSVEIEWELQKENSKRWNPEIQYTSNYNKSINVDFTVDTNGVYSEPRPIGTRYLTRNL

SEQ ID NO: 41 - DNA, 2238 bp, synthetic construct
  misc_feature 1..2238: note = synthetically generated sequence
  source 1..2238: mol_type = other DNA
atggctgccgatggttatcttccagattggctcgaggacactctctctgaaggaataagacagtggtggaagctcaaacctggcccaccaccaccaaagcccgcagagcggcataaggacgacagcaggggtcttgtgcttcctgggtacaagtacctcggacccttcaacggactcgacaagggagagccggtcaacgccgcagacgccgcggccctcgagcacgacaaagcctacgaccggcagctcgacagcggagacaacccgtacctcaagtacaaccacgccgacgcggagtttcaggagcgccttaaagaagatacgtcttttgggggcaacctcggacgagcagtcttccaggcgaaaaagagggttcttgaacctctgggcctggttgaggaacctgttaagacggctccgggaaaaaagaggccggtagagcactctcctgtggagccagactcctcctcgggaaccggaaaggcgggccagcagcctgcaagaaaaagattgaattttggtcagactggagacgcagactcagtacctgacccccagcctctcggacagccaccagcagccccctctggtctgggaactaatacgatggctacaggcagtggcgcaccaatggcagacaataacgagggcgccgacggagtgggtaattcctcgggaaattggcattgcgattccacatggatgggcgacagagtcatcaccaccagcacccgaacctgggccctgcccacctacaacaaccacctctacaaacaaatttccagccaatcaggagcctcgaacgacaatcactactttggctacagcaccccttgggggtattttgacttcaacagattccactgccacttttcaccacgtgactggcaaagactcatcaacaacaactggggattccgacccaagagactcaacttcaagctctttaacattcaagtcaaagaggtcacgcagaatgacggtacgacgacgattgccaataaccttaccagcacggttcaggtgtttactgactcggagtaccagctcccgtacgtcctcggctcggcgcatcaaggatgcctcccgccgttcccagcagacgtcttcatggtgccacagtatggatacctcaccctgaacaacgggagtcaggcagtaggacgctcttcattttactgcctggagtactttccttctcagatgctgcgtaccggaaacaactttaccttcagctacacttttgaggacgttcctttccacagcagctacgctcacagccagagtctggaccgtctcatgaatcctctcatcgaccagtacctgtattacttgagcagaacaaacactccaagtggaaccaccacgcagtcaaggcttcagttttctcaggccggagcgagtgacattcgggaccagtctaggaactggcttcctggaccctgttaccgccagcagcgagtatcaaagacatctgcggataacaacaacagtgaatactcgtggactggagctaccaagtaccacctcaatggcagagactctctggtgaatccgggcccggccatggcaagccacaaggacgatgaagaaaagttttttcctcagagcggggttctcatctttgggaagcaaggctcagagaaaacaaatgtggacattgaaaaggtcatgattacagacgaagaggaaatcaggacaaccaatcccgtggctacggagcagtatggttctgtatctaccaacctccagggaggcaacctagcaaaccaagactacacaaaaactgctaggcaagcagctaccgcagatgtcaacacacaaggcgttcttccaggcatggtctggcaggacagagatgtgtaccttcaggggcccatctgggcaaagattccacacacggacggacattttcacccctctcccctcatgggtggattcggacttaaacaccctcctccccagattctcatcaagaacaccccggtacctgcgaatccttcgaccaccttctgtgcggcaaagtttgcttccttcatcacacagtactccacgggacaggtcagcgtggagatcgagtgggagctgcagaaggaaaacagcaaacgctggaatcccgaaattcagtacacttccaactacaacaagtctattaatgtggactttactgtggacactaatggcgtgtattcagagcctcgccccattggcaccagatacctgactcgtaatctgtaa

SEQ ID NO: 42 - protein, 745 aa, synthetic construct
  REGION 1..745: note = synthetically generated sequence
MAADGYLPDWLEDTLSEGIRQWWKLKPGPPPPKPAERHKDDSRGLVLPGYKYLGPFNGLDKGEPVNAADAAALEHDKAYDRQLDSGDNPYLKYNHADAEFQERLKEDTSFGGNLGRAVFQAKKRVLEPLGLVEEPVKTAPGKKRPVEHSPVEPDSSSGTGKAGQQPARKRLNFGQTGDADSVPDPQPLGQPPAAPSGLGTNTMATGSGAPMADNNEGADGVGNSSGNWHCDSTWMGDRVITTSTRTWALPTYNNHLYKQISSQSGASNDNHYFGYSTPWGYFDFNRFHCHFSPRDWQRLINNNWGFRPKRLNFKLFNIQVKEVTQNDGTTTIANNLTSTVQVFTDSEYQLPYVLGSAHQGCLPPFPADVFMVPQYGYLTLNNGSQAVGRSSFYCLEYFPSQMLRTGNNFTFSYTFEDVPFHSSYAHSQSLDRLMNPLIDQYLYYLSRTNTPSGTTTQSRLQFSQAGASDIRDQSRNWLPGPCYRQQRVSKTSADNNNSEYSWTGATKYHLNGRDSLVNPGPAMASHKDDEEKFFPQSGVLIFGKQGSEKTNVDIEKVMITDEEEIRTTNPVATEQYGSVSTNLQGGNLANQDYTKTARQAATADVNTQGVLPGMVWQDRDVYLQGPIWAKIPHTDGHFHPSPLMGGFGLKHPPPQILIKNTPVPANPSTTFCAAKFASFITQYSTGQVSVEIEWELQKENSKRWNPEIQYTSNYNKSINVDFTVDTNGVYSEPRPIGTRYLTRNL

SEQ ID NO: 43 - DNA, 2238 bp, synthetic construct
  misc_feature 1..2238: note = synthetically generated sequence
  source 1..2238: mol_type = other DNA
atggctgccgatggttatcttccagattggctcgaggacactctctctgaaggaataagacagtggtggaagctcaaacctggcccaccaccaccaaagcccgcagagcggcataaggacgacagcaggggtcttgtgcttcctgggtacaagtacctcggacccttcaacggactcgacaagggagagccggtcaacgaggcagacgccgcggccctcgagcacgacaaagcctacgaccggcagctcgacagcggagacaacccgtacctcaagtacaaccacgccgacgcggagtttcaggagcgccttaaagaagatacgtcttttgggggcaacctcggacgagcagtcttccaggcgaaaaagagggttcttgaacctctgggcctggttgaggaacctgttaagacggctccgggaaaaaagaggccggtagagcactctcctgtggagccagactcctcctcgggaaccggaaaggcgggccagcagcctgcaagaaaaagattgaattttggtcagactggagacgcagactcagtacctgacccccagcctctcggacagccaccagcagccccctctggtctgggaactaatacgatggctacaggcagtggcgcaccaatggcagacaataacgagggcgccgacggagtgggtaattcctcgggaaattggcattgcgattccacatggatgggcgacagagtcatcaccaccagcacccgaacctgggccctgcccacctacaacaaccacctctacaaacaaatttccagccaatcaggagcctcgaacgacaatcactactttggctacagcaccccttgggggtattttgacttcaacagattccactgccacttttcaccacgtgactggcaaagactcatcaacaacaactggggattccgacccaagagactcaacttcaagctctttaacattcaagtcaaagaggtcacgcagaatgacggtacgacgacgattgccaataaccttaccagcacggttcaggtgtttactgactcggagtaccagctcccgtacgtcctcggctcggcgcatcaaggatgcctcccgccgttcccagcagacgtcttcatggtgccacagtatggatacctcaccctgaacgacgggagtcaggcagtaggacgctcttcattttactgcctggagtactttccttctcagatgctgcgtaccggaaacaactttaccttcagctacacttttgaggacgttcctttccacagcagctacgctcacagccagagtctggaccgtctcatgaatcctctcatcgaccagtacctgtattacttgagcagaacaaacactccaagtggaaccaccacgcagtcaaggcttcagttttctcaggccggagcgagtgacattcgggaccagtctaggaactggcttcctggaccctgttaccgccagcagcgagtatcaaagacatctgcggataacaacaacagtgaatactcgtggactggagctaccaagtaccacctcaatggcagagactctctggtgaatccgggcccggccatggcaagccacaaggacgatgaagaaaagttttttcctcagagcggggttctcatctttgggaagcaaggctcagagaaaacaaatgtggacattgaaaaggtcatgattacagacgaagaggaaatcaggacaaccaatcccgtggctacggagcagtatggttctgtatctaccaacctccagagaggcaacctagcagaccaagactacacaaaaactgctaggcaagcagctaccgcagatgtcaacacacaaggcgttcttccaggcatggtctggcaggacagagatgtgtaccttcaggggcccatctgggcaaagattccacacacggacggacattttcacccctctcccctcatgggtggattcggacttaaacaccctcctccccagattctcatcaagaacaccccggtacctgcgaatccttcgaccaccttcagtgcggcaaagtttgcttccttcatcacacagtactccacgggacaggtcagcgtggagatcgagtgggagctgcagaaggaaaacagcaaacgctggaatcccgaaattcagtacacttccaactacaacaagtctattaatgtggactttactgtggacactaatggcgtgtattcagagcctcgccccattggcaccagatacctgactcgtaatctgtaa

SEQ ID NO: 44 - protein, 745 aa, synthetic construct
  REGION 1..745: note = synthetically generated sequence
MAADGYLPDWLEDTLSEGIRQWWKLKPGPPPPKPAERHKDDSRGLVLPGYKYLGPFNGLDKGEPVNEADAAALEHDKAYDRQLDSGDNPYLKYNHADAEFQERLKEDTSFGGNLGRAVFQAKKRVLEPLGLVEEPVKTAPGKKRPVEHSPVEPDSSSGTGKAGQQPARKRLNFGQTGDADSVPDPQPLGQPPAAPSGLGTNTMATGSGAPMADNNEGADGVGNSSGNWHCDSTWMGDRVITTSTRTWALPTYNNHLYKQISSQSGASNDNHYFGYSTPWGYFDFNRFHCHFSPRDWQRLINNNWGFRPKRLNFKLFNIQVKEVTQNDGTTTIANNLTSTVQVFTDSEYQLPYVLGSAHQGCLPPFPADVFMVPQYGYLTLNDGSQAVGRSSFYCLEYFPSQMLRTGNNFTFSYTFEDVPFHSSYAHSQSLDRLMNPLIDQYLYYLSRTNTPSGTTTQSRLQFSQAGASDIRDQSRNWLPGPCYRQQRVSKTSADNNNSEYSWTGATKYHLNGRDSLVNPGPAMASHKDDEEKFFPQSGVLIFGKQGSEKTNVDIEKVMITDEEEIRTTNPVATEQYGSVSTNLQRGNLADQDYTKTARQAATADVNTQGVLPGMVWQDRDVYLQGPIWAKIPHTDGHFHPSPLMGGFGLKHPPPQILIKNTPVPANPSTTFSAAKFASFITQYSTGQVSVEIEWELQKENSKRWNPEIQYTSNYNKSINVDFTVDTNGVYSEPRPIGTRYLTRNL

SEQ ID NO: 45 - DNA, 2238 bp, synthetic construct
  misc_feature 1..2238: note = synthetically generated sequence
  source 1..2238: mol_type = other DNA
atggctgccgatggttatcttccagattggctcgaggacactctctctgaaggaataagacagtggtggaagctcaaacctggcccaccaccaccaaagcccgcagagcggcataaggacgacagcaggggtcttgtgcttcctgggtacaagtacctcggacccttcaacggactcgacaagggagagccggtcaacgccgcagacgccgcggccctcgagcacgacaaagcctacgaccggcagctcgacagcggagacaacccgtacctcaagtacaaccacgccgacgcggagtttcaggagcgccttaaagaagatacgtcttttgggggcaacctcggacgagcagtcttccaggcgaaaaagagggttcttgaacctctgggcctggttgaggaacctgttaagacggctccgggaaaaaagaggccggtagagcactctcctgtggagccagactcctcctcgggaaccggaaaggcgggccagcagcctgcaagaaaaagattgaattttggtcagactggagacgcagactcagtacctgacccccagcctctcggacagccaccagcagccccctctggtctgggaactaatacgatggctacaggcagtggcgcaccaatggcagacaataacgagggcgccgacggagtgggtaattcctcgggaaattggcattgcgattccacatggatgggcgacagagtcatcaccaccagcacccgaacctgggccctgcccacctacaacaaccacctctacaaacaaatttccagccaatcaggagcctcgaacgacaatcactactttggctacagcaccccttgggggtattttgacttcaacagattccactgccacttttcaccacgtgactggcaaagactcatcaacaacaactggggattccgacccaagagactcaacttcaagctctttaacattcaagtcaaagaggtcacgcagaatgacggtacgacgacgattgccaataaccttaccagcacggttcaggtgtttactgactcggagtaccagctcccgtacgtcctcggctcggcgcatcaaggatgcctcccgccgttcccagcagacgtcttcatggtgccacagtatggatacctcaccctgaacaacgggagtcaggcagtaggacgctcttcattttactgcctggagtactttccttctcagatgctgcgtaccggaaacaactttaccttcagctacacttttgaggacgttcctttccacagcagctacgctcacagccagagtctggaccgtctcatgaatcctctcatcgaccagtacctgtattacttgagcagaacaaacactccaagtggaaccaccacgcagtcaaggcttcagttttctcaggccggagcgagtgacattcgggaccagtctaggaactggcttcctggaccctgttaccgccagcagcgagtatcaaagacatctgcggataacaacaacagtgaatactcgtggactggagctaccaagtaccacctcaatggcagagactctctggtgaatccgggcccggccatggcaagccacaaggacgatgaagaaaagttttttcctcagagcggggttctcatctttgggaagcaaggctcagagaaaacaaatgtggacattgaaaaggtcatgattacagacgaagaggaaatcaggacaaccaatcccgtggctacggagcagtatggttctgtatctaccaacctccagagaggcaacctagcaaaccaagactacacaaaaactgctaggcaagcagctaccgcagatgtcaacacacaaggcgttcttccaggcatggtctggcaggacagagatgtgtaccttcaggggcccatctgggcaaagattccacacacggacggacattttcacccctctcccctcatgggtggattcggacttaaacaccctcctccccagattctcatcaagaacaccccggtacctgcgaatccttcgaccaccttcagtgcggcaaagtttgcttccttcatcacacagtactccacgggacaggtcagcgtggagatcgagtgggagctgcagaaggaaaacagcaaacgctggaatcccgaaattcagtacacttccaactacaacaagtctattaatgtggactttactgtggacactaatggcgtgtattcagagcctcgccccattggcaccagatacctgactcgtaatctgtaa

SEQ ID NO: 46 - protein, 745 aa, synthetic construct
  REGION 1..745: note = synthetically generated sequence
MAADGYLPDWLEDTLSEGIRQWWKLKPGPPPPKPAERHKDDSRGLVLPGYKYLGPFNGLDKGEPVNAADAAALEHDKAYDRQLDSGDNPYLKYNHADAEFQERLKEDTSFGGNLGRAVFQAKKRVLEPLGLVEEPVKTAPGKKRPVEHSPVEPDSSSGTGKAGQQPARKRLNFGQTGDADSVPDPQPLGQPPAAPSGLGTNTMATGSGAPMADNNEGADGVGNSSGNWHCDSTWMGDRVITTSTRTWALPTYNNHLYKQISSQSGASNDNHYFGYSTPWGYFDFNRFHCHFSPRDWQRLINNNWGFRPKRLNFKLFNIQVKEVTQNDGTTTIANNLTSTVQVFTDSEYQLPYVLGSAHQGCLPPFPADVFMVPQYGYLTLNNGSQAVGRSSFYCLEYFPSQMLRTGNNFTFSYTFEDVPFHSSYAHSQSLDRLMNPLIDQYLYYLSRTNTPSGTTTQSRLQFSQAGASDIRDQSRNWLPGPCYRQQRVSKTSADNNNSEYSWTGATKYHLNGRDSLVNPGPAMASHKDDEEKFFPQSGVLIFGKQGSEKTNVDIEKVMITDEEEIRTTNPVATEQYGSVSTNLQRGNLANQDYTKTARQAATADVNTQGVLPGMVWQDRDVYLQGPIWAKIPHTDGHFHPSPLMGGFGLKHPPPQILIKNTPVPANPSTTFSAAKFASFITQYSTGQVSVEIEWELQKENSKRWNPEIQYTSNYNKSINVDFTVDTNGVYSEPRPIGTRYLTRNL

SEQ ID NO: 47 - DNA, 2238 bp, synthetic construct
  misc_feature 1..2238: note = synthetically generated sequence
  source 1..2238: mol_type = other DNA
atggctgccgatggttatcttccagattggctcgaggacactctctctgaaggaataagacagtggtggaagctcaaacctggcccaccaccaccaaagcccgcagggcggcataaggacgacagcaggggtcttgtgcttcctgggtacaagtacctcggacccttcaacggactcgacaagggagagccggtcaacgaggcagacgccgcggccctcgagcacgacaaagcctacgaccggcagctcgacagcggagacaacccgtacctcaagtacaaccacgccgacgcggagtttcaggagcgccttaaagaagatacgtcttttgggggcaacctcggacgagcagtcttccaggcgaaaaagagggttcttgaacctctgggcctggttgaggaacctgttaagacggctccgggaaaaaagaggccggtagagcactctcctgtggagccagactcctcctcgggaaccggaaaggcgggccagcagcctgcaagaaaaagattgaattttggtcagactggagacgcagactcagtacctgacccccagcctctcggacagccaccagcagccccctctggtctgggaactaatacgatggctacaggcagtggcgcaccaatggcagacaataacgagggcgccgacggagtgggtaattcctcgggaaattggcattgcgattccacatggatgggcgacagagtcatcaccaccagcacccgaacctgggccctgcccacctacaacaaccacctctacaaacaaatttccagccaatcaggagcctcgaacgacaatcactactttggctacagcaccccttgggggtattttgacttcaacagattccactgccacttttcaccacgtgactggcaaagactcatcaacaacaactggggattccgacccaagagactcaacttcaagctctttaacattcaagtcaaagaggtcacgcagaatgacggtacgacgacgattgccaataaccttaccagcacggttcaggtgtttactgactcggagtaccagctcccgtacgtcctcggctcggcgcatcaaggatgcctcccgccgttcccagcagacgtcttcatggtgccacagtatggatacctcaccctgaacaacgggagtcaggcagtaggacgctcttcattttactgcctggagtactttccttctcagatgctgcgtaccggaaacagctttaccttcagctacacttttgaggacgttcctttccacagcagctacgctcacagccagagtctggaccgtctcatgaatcctctcatcgaccagtacctgtattacttgagcagaacaaacactccaagtggaaccaccacgcagtcaaggcttcagttttctcaggccggagcgagtgacattcgggaccagtctaggaactggcttcctggaccctgttaccgccagcagcgagtatcaaagacatctgcggataacaacaacagtgaatactcgtggactggagctaccaagtaccacctcaatggcagagactctctggtgaatccgggcccggccatggcaagccacaaggacgatgaagaaaagttttttcctcagagcggggttctcatctttgggaagcaaggctcagagaaaacaaatgtggacattgaaaaggtcatgattacagacgaagaggaaatcaggacaaccaatcccgtggctacggagcagtatggttctgtatctaccaacctccagagaggcaacctagcagaccaagactacacaaaaactgctaggcaagcagctaccgcagatgtcaacacacaaggcgttcttccaggcatggtctggcaggacagagatgtgtaccttcaggggcccatctgggcaaagattccacacacggacggacattttcacccctctcccctcatgggtggattcggacttaaacaccctcctccccagattctcatcaagaacaccccggtacctgcgaatccttcgaccaccttcagtgcggcaaagtttgcttccttcatcacacagtactccacgggacaggtcagcgtggagatcgagtgggagctgcagaaggaaaacagcaaacgctggaatcccgaaattcagtacacttccaactacaacaagtctattaatgtggactttactgtggacactaatggcgtgtattcagagcctcgccccattggcaccagatacctgactcgtaatctgtaa

SEQ ID NO: 48 - protein, 745 aa, synthetic construct
  REGION 1..745: note = synthetically generated sequence
MAADGYLPDWLEDTLSEGIRQWWKLKPGPPPPKPAGRHKDDSRGLVLPGYKYLGPFNGLDKGEPVNEADAAALEHDKAYDRQLDSGDNPYLKYNHADAEFQERLKEDTSFGGNLGRAVFQAKKRVLEPLGLVEEPVKTAPGKKRPVEHSPVEPDSSSGTGKAGQQPARKRLNFGQTGDADSVPDPQPLGQPPAAPSGLGTNTMATGSGAPMADNNEGADGVGNSSGNWHCDSTWMGDRVITTSTRTWALPTYNNHLYKQISSQSGASNDNHYFGYSTPWGYFDFNRFHCHFSPRDWQRLINNNWGFRPKRLNFKLFNIQVKEVTQNDGTTTIANNLTSTVQVFTDSEYQLPYVLGSAHQGCLPPFPADVFMVPQYGYLTLNNGSQAVGRSSFYCLEYFPSQMLRTGNSFTFSYTFEDVPFHSSYAHSQSLDRLMNPLIDQYLYYLSRTNTPSGTTTQSRLQFSQAGASDIRDQSRNWLPGPCYRQQRVSKTSADNNNSEYSWTGATKYHLNGRDSLVNPGPAMASHKDDEEKFFPQSGVLIFGKQGSEKTNVDIEKVMITDEEEIRTTNPVATEQYGSVSTNLQRGNLADQDYTKTARQAATADVNTQGVLPGMVWQDRDVYLQGPIWAKIPHTDGHFHPSPLMGGFGLKHPPPQILIKNTPVPANPSTTFSAAKFASFITQYSTGQVSVEIEWELQKENSKRWNPEIQYTSNYNKSINVDFTVDTNGVYSEPRPIGTRYLTRNL

SEQ ID NO: 49 - DNA, 2238 bp, synthetic construct
  misc_feature 1..2238: note = synthetically generated sequence
  source 1..2238: mol_type = other DNA
atggctgccgatggttatcttccagattggctcgaggacactctctctgaaggaataagacagtggtggaagctcaaacctggcccaccaccaccaaagcccgcagggcggcataaggacgacagcaggggtcttgtgcttcctgggtacaagtacctcggacccttcaacggactcgacaagggagagccggtcaacgaggcagacgccgcggccctcgagcacgacaaagcctacgaccggcagctcgacagcggagacaacccgtacctcaagtacaaccacgccgacgcggagtttcaggagcgccttaaagaagatacgtcttttgggggcaacctcggacgagcagtcttccaggcgaaaaagagggttcttgaacctctgggcctggttgaggaacctgttaagacggctccgggaaaaaagaggccggtagagcactctcctgtggagccagactcctcctcgggaaccggaaaggcgggccagcagcctgcaagaaaaagattgaattttggtcagactggagacgcagactcagtacctgacccccagcctctcggacagccaccagcagccccctctggtctgggaactaatacgatggctacaggcagtggcgcaccaatggcagacaataacgagggcgccgacggagtgggtaattcctcgggaaattggcattgcgattccacatggatgggcgacagagtcatcaccaccagcacccgaacctgggccctgcccacctacaacaaccacctctacaaacaaatttccagccaatcaggagcctcgaacgacaatcactactttggctacagcaccccttgggggtattttgacttcaacagattccactgccacttttcaccacgtgactggcaaagactcatcaacaacaactggggattccgacccaagagactcaacttcaagctctttaacattcaagtcaaagaggtcacgcagaatgacggtacgacgacgattgccaataagcttaccagcacggttcaggtgtttactgactcggagtaccagctcccgtacgtcctcggctcggcgcatcaaggatgcctcccgccgttcccagcagacgtcttcatggtgccacagtatggatacctcaccctgaacaacgggagtcaggcagtaggacgctcttcattttactgcctggagtactttccttctcagatgctgcgtaccggaaacagctttaccttcagctacacttttgaggacgttcctttccacagcagctacgctcacagccagagtctggaccgtctcatgaatcctctcatcgaccagtacctgtattacttgagcagaacaaacactccaagtggaaccaccacgcagtcaaggcttcagttttctcaggccggagcgagtgacattcgggaccagtctaggaactggcttcctggaccctgttaccgccagcagcgagtatcaaagacatctgcggataacaacaacagtgaatactcgtggactggagctaccaagtaccacctcaatggcagagactctctggtgaatccgggcccggccatggcaagccacaaggacgatgaagaaaagttttttcctcagagcggggttctcatctttgggaagcaaggctcagagaaaacaaatgtggacattgaaaaggtcatgattacagacgaagaggaaatcaggacaaccaatcccgtggctacggagcagtatggttctgtatctaccaacctccagagaggcaacctagcaaaccaagactacacaaaaactgctaggcaagcagctaccgcagatgtcaacacacaaggcgttcttccaggcatggtctggcaggacagagatgtgtaccttcaggggcccatctgggcaaagattccacacacggacggacattttcacccctctcccctcatgggtggattcggacttaaacaccctcctccccagattctcatcaagaacaccccggtacctgcgaatccttcgaccaccttcagtgcggcaaagtttgcttccttcatcacacagtactccacgggacaggtcagcgtggagatcgagtgggagctgcagaaggaaaacagcaaacgctggaatcccgaaattcagtacacttccaactacaacaagtctattaatgtggactttactgtggacactaatggcgtgtattcagagcctcgccccattggcaccagatacctgactcgtaatctgtaa

SEQ ID NO: 50 - protein, 745 aa, synthetic construct
  REGION 1..745: note = synthetically generated sequence
MAADGYLPDWLEDTLSEGIRQWWKLKPGPPPPKPAGRHKDDSRGLVLPGYKYLGPFNGLDKGEPVNEADAAALEHDKAYDRQLDSGDNPYLKYNHADAEFQERLKEDTSFGGNLGRAVFQAKKRVLEPLGLVEEPVKTAPGKKRPVEHSPVEPDSSSGTGKAGQQPARKRLNFGQTGDADSVPDPQPLGQPPAAPSGLGTNTMATGSGAPMADNNEGADGVGNSSGNWHCDSTWMGDRVITTSTRTWALPTYNNHLYKQISSQSGASNDNHYFGYSTPWGYFDFNRFHCHFSPRDWQRLINNNWGFRPKRLNFKLFNIQVKEVTQNDGTTTIANKLTSTVQVFTDSEYQLPYVLGSAHQGCLPPFPADVFMVPQYGYLTLNNGSQAVGRSSFYCLEYFPSQMLRTGNSFTFSYTFEDVPFHSSYAHSQSLDRLMNPLIDQYLYYLSRTNTPSGTTTQSRLQFSQAGASDIRDQSRNWLPGPCYRQQRVSKTSADNNNSEYSWTGATKYHLNGRDSLVNPGPAMASHKDDEEKFFPQSGVLIFGKQGSEKTNVDIEKVMITDEEEIRTTNPVATEQYGSVSTNLQRGNLANQDYTKTARQAATADVNTQGVLPGMVWQDRDVYLQGPIWAKIPHTDGHFHPSPLMGGFGLKHPPPQILIKNTPVPANPSTTFSAAKFASFITQYSTGQVSVEIEWELQKENSKRWNPEIQYTSNYNKSINVDFTVDTNGVYSEPRPIGTRYLTRNL

SEQ ID NO: 51 - DNA, 2238 bp, synthetic construct; identical to SEQ ID NO: 17
  misc_feature 1..2238: note = synthetically generated sequence
  source 1..2238: mol_type = other DNA

SEQ ID NO: 52 - protein, 745 aa, synthetic construct; identical to SEQ ID NO: 18
  REGION 1..745: note = synthetically generated sequence

SEQ ID NO: 53 - DNA, 2238 bp, synthetic construct
  misc_feature 1..2238: note = synthetically generated sequence
  source 1..2238: mol_type = other DNA
atggctgccgatggttatcttccagattggctcgaggacactctctctgaaggaataagacagtggtggaagctcaaacctggcccaccaccaccaaagcccgcagagcggcataaggacgacagcaggggtcttgtgcttcctgggtacaagtacctcggacccttcaacggactcgacaagggagagccggtcaacgaggcagacgccgcggccctcgagcacgacaaagcctacgaccggcagctcgacagcggagacaacccgtacctcaagtacaaccacgccgacgcggagtttcaggagcgccttaaagaagatacgtcttttgggggcaacctcggacgagcagtcttccaggcgaaaaagagggttcttgaacctctgggcctggttgaggaacctgttaagacggctccgggaaaaaagaggccggtagagcactctcctgtggagccagactcctcctcgggaaccggaaaggcgggccagcagcctgcaagaaaaagattgaattttggtcagactggagacgcagactcagtacctgacccccagcctctcggacagccaccagcagccccctctggtctgggaactaatacgatggctacaggcagtggcgcaccaatggcagacaataacgagggcgccgacggagtgggtaattcctcgggaaattggcattgcgattccacatggatgggcgacagagtcatcaccaccagcacccgaacctgggccctgcccacctacaacaaccacctctacaaacaaatttccagccaatcaggagcctcgaacgacaatcactactttggctacagcaccccttgggggtattttgacttcaacagattccactgccacttttcaccacgtgactggcaaagactcatcaacaacaactggggattccgacccaagagactcaacttcaagctctttaacattcaagtcaaagaggtcacgcagaatgacggtacgacgacgattgccaataaccttaccagcacggttcaggtgtttactgactcggagtaccagctcccgtacgtcctcggctcggcgcatcaaggatgcctcccgccgttcccagcagacgtcttcatggtgccacagtatggatacctcaccctgaacaacgggagtcaggcagtaggacgctcttcattttactgcctggagtactttccttctcagatgctgcgtaccggaaacaactttaccttcagctacacttttgaggacgttcctttccacagcaactacgctcacagccagagtctggaccgtctcatgaatcctctcatcgaccagtacctgtattacttgagcagaacaaacactccaagtggaaccaccacgcagtcaaggcttcagttttctcaggccggagcgagtgacattcgggaccagtctaggaactggcttcctggaccctgttaccgccagcagcgagtatcaaagacatctgcggataacaacaacagtgaatactcgtggactggagctaccaagtaccacctcaatggcagagactctctggtgaatccgggcccggccatggcaagccacaaggacgatgaagaaaagttttttcctcagagcggggttctcatctttgggaagcaaggctcagagaaaacaaatgtggacattgaaaaggtcatgattacagacgaagaggaaatcaggacaaccaatcccgtggctacggagcagtatggttctgtatctaccaacctccagagaggcaacctagcaatctccgaccagacaaaacacgctaggcaagcagctaccgcagatgtcaacacacaaggcgttcttccaggcatggtctggcaggacagagatgtgtaccttcaggggcccatctgggcaaagattccacacacggacggacattttcacccctctcccctcatgggtggattcggacttaaacaccctcctccccagattctcatcaagaacaccccggtacctgcgaatccttcgaccaccttcagtgcggcaaagtttgcttccttcatcacacagtactccacgggacaggtcagcgtggagatcgagtgggagctgcagaaggaaaacagcaaacgctggaatcccgaaattcagtacacttccaactacaacaagtctattaatgtggactttactgtggacactaatggcgtgtattcagagcctcgccccattggcaccagatacctgactcgtaatctgtaa

SEQ ID NO: 54 - protein, 745 aa, synthetic construct
  REGION 1..745: note = synthetically generated sequence
MAADGYLPDWLEDTLSEGIRQWWKLKPGPPPPKPAERHKDDSRGLVLPGYKYLGPFNGLDKGEPVNEADAAALEHDKAYDRQLDSGDNPYLKYNHADAEFQERLKEDTSFGGNLGRAVFQAKKRVLEPLGLVEEPVKTAPGKKRPVEHSPVEPDSSSGTGKAGQQPARKRLNFGQTGDADSVPDPQPLGQPPAAPSGLGTNTMATGSGAPMADNNEGADGVGNSSGNWHCDSTWMGDRVITTSTRTWALPTYNNHLYKQISSQSGASNDNHYFGYSTPWGYFDFNRFHCHFSPRDWQRLINNNWGFRPKRLNFKLFNIQVKEVTQNDGTTTIANNLTSTVQVFTDSEYQLPYVLGSAHQGCLPPFPADVFMVPQYGYLTLNNGSQAVGRSSFYCLEYFPSQMLRTGNNFTFSYTFEDVPFHSNYAHSQSLDRLMNPLIDQYLYYLSRTNTPSGTTTQSRLQFSQAGASDIRDQSRNWLPGPCYRQQRVSKTSADNNNSEYSWTGATKYHLNGRDSLVNPGPAMASHKDDEEKFFPQSGVLIFGKQGSEKTNVDIEKVMITDEEEIRTTNPVATEQYGSVSTNLQRGNLAISDQTKHARQAATADVNTQGVLPGMVWQDRDVYLQGPIWAKIPHTDGHFHPSPLMGGFGLKHPPPQILIKNTPVPANPSTTFSAAKFASFITQYSTGQVSVEIEWELQKENSKRWNPEIQYTSNYNKSINVDFTVDTNGVYSEPRPIGTRYLTRNL

SEQ ID NO: 55 - DNA, 2238 bp, synthetic construct
  misc_feature 1..2238: note = synthetically generated sequence
  source 1..2238: mol_type = other DNA
atggctgccgatggttatcttccagattggctcgaggacactctctctgaaggaataagacagtggtggaagctcaaacctggcccaccaccaccaaagcccgcagagcggcataaggacgacagcaggggtcttgtgcttcctgggtacaagtacctcggacccttcaacggactcgacaagggagagccggtcaacgaggcagacgccgcggccctcgagcacgacaaagcctacgaccggcagctcgacagcggagacaacccgtacctcaagtacaaccacgccgacgcggagtttcaggagcgccttaaagaagatacgtcttttgggggcaacctcggacgagcagtcttccaggcgaaaaagagggttcttgaacctctgggcctggttgaggaacctgttaagacggctccgggaaaaaagaggccggtagagcactctcctgtggagccagactcctcctcgggaaccggaaaggcgggccagcagcctgcaagaaaaagattgaattttggtcagactggagacgcagactcagtacctgacccccagcctctcggacagccaccagcagccccctctggtctgggaactaatacgatggctacaggcagtggcgcaccaatggcagacgataacgagggcgccgacggagtgggtaattcctcgggaaattggcattgcgattccacatggatgggcgacagagtcatcaccaccagcacccgaacctgggccctgcccacctacaacaaccacctctacaaacaaatttccagccaatcaggagcctcgaacgacaatcactactttggctacagcaccccttgggggtattttgacttcaacagattccactgccacttttcaccacgtgactggcaaagactcatcaacaacaactggggattccgacccaagagactcaacttcaagctctttaacattcaagtcaaagaggtcacgcagaatgacggtacgacgacgattgccaataaccttaccagcacggttcaggtgtttactgactcggagtaccagctcccgtacgtcctcggctcggcgcatcaaggatgcctcccgccgttcccagcagacgtcttcatggtgccacagtatggatacctcaccctgaacaacgggagtcaggcagtaggacgctcttcattttactgcctggagtactttccttctcagatgctgcgtaccggaaacaactttaccttcagctacacttttgaggacgttcctttccacagcagctacgctcacagccagagtctggaccgtctcatgaatcctctcatcgaccagtacctgtattacttgagcagaacaaacactccaagtggaaccaccacgcagtcaaggcttcagttttctcaggccggagcgagtgacattcgggaccagtctaggaactggcttcctggaccctgttaccgccagcagcgagtatcaaagacatctgcggataacaacaacagtgaatactcgtggactggagctaccaagtaccacctcaatggcagagactctctggtgaatccgggcccggccatggcaagccacaaggacgatgaagaaaagttttttcctcagagcggggttctcatctttgggaagcaaggctcagagaaaacaaatgtggacattgaaaaggtcatgattacagacgaagaggaaatcaggacaaccaatcccgtggctacggagcagtatggttctgtatctaccaacctccagagaggcaacctagcaatctccgaccagacaaaacacgctaggcaagcagctaccgcagatgtcaacacacaaggcgttcttccaggcatggtctggcaggacagagatgtgtaccttcaggggcccatctgggcaaagattccacacacggacggacattttcacccctctcccctcatgggtggattcggacttaaacaccctcctccccagattctcatcaagaacaccccggtacctgcgaatccttcgaccaccttcagtgcggcaaagtttgcttccttcatcacacagtactccacgggacaggtcagcgtggagatcgagtgggagctgcagaaggaaaacagcaaacgctggaatcccgaaattcagtacacttccaactacaacaagtctattaatgtggactttactgtggacactaatggcgtgtattcagagcctcgccccattggcaccagatacctgactcgtaatctgtaa

SEQ ID NO: 56 - protein, 745 aa, synthetic construct
  REGION 1..745: note = synthetically generated sequence
MAADGYLPDWLEDTLSEGIRQWWKLKPGPPPPKPAERHKDDSRGLVLPGYKYLGPFNGLDKGEPVNEADAAALEHDKAYDRQLDSGDNPYLKYNHADAEFQERLKEDTSFGGNLGRAVFQAKKRVLEPLGLVEEPVKTAPGKKRPVEHSPVEPDSSSGTGKAGQQPARKRLNFGQTGDADSVPDPQPLGQPPAAPSGLGTNTMATGSGAPMADDNEGADGVGNSSGNWHCDSTWMGDRVITTSTRTWALPTYNNHLYKQISSQSGASNDNHYFGYSTPWGYFDFNRFHCHFSPRDWQRLINNNWGFRPKRLNFKLFNIQVKEVTQNDGTTTIANNLTSTVQVFTDSEYQLPYVLGSAHQGCLPPFPADVFMVPQYGYLTLNNGSQAVGRSSFYCLEYFPSQMLRTGNNFTFSYTFEDVPFHSSYAHSQSLDRLMNPLIDQYLYYLSRTNTPSGTTTQSRLQFSQAGASDIRDQSRNWLPGPCYRQQRVSKTSADNNNSEYSWTGATKYHLNGRDSLVNPGPAMASHKDDEEKFFPQSGVLIFGKQGSEKTNVDIEKVMITDEEEIRTTNPVATEQYGSVSTNLQRGNLAISDQTKHARQAATADVNTQGVLPGMVWQDRDVYLQGPIWAKIPHTDGHFHPSPLMGGFGLKHPPPQILIKNTPVPANPSTTFSAAKFASFITQYSTGQVSVEIEWELQKENSKRWNPEIQYTSNYNKSINVDFTVDTNGVYSEPRPIGTRYLTRNL

SEQ ID NO: 57 - DNA, 2238 bp, synthetic construct; identical to SEQ ID NO: 17
  misc_feature 1..2238: note = synthetically generated sequence
  source 1..2238: mol_type = other DNA

SEQ ID NO: 58 - protein, 745 aa, synthetic construct; identical to SEQ ID NO: 18
  REGION 1..745: note = synthetically generated sequence

SEQ ID NO: 59 - DNA, 2238 bp, synthetic construct
  misc_feature 1..2238: note = synthetically generated sequence
  source 1..2238: mol_type = other DNA
atggctgccgatggttatcttccagattggctcgaggacactctctctgaaggaataagacagtggtggaagctcaaacctggcccaccaccaccaaagcccgcagagcggcataaggacgacagcaggggtcttgtgcttcctgggtacaagtacctcggacccttcaacggactcgacaagggagagccggtcaacgccgcagacgccgcggccctcgagcacgacaaagcctacgaccggcagctcgacagcggagacaacccgtacctcaagtacaaccacgccgacgcggagtttcaggagcgccttaaagaagatacgtcttttgggggcaacctcggacgagcagtcttccaggcgaaaaagagggttcttgaacctctgggcctggttgaggaacctgttaagacggctccgggaaaaaagaggccggtagagcactctcctgtggagccagactcctcctcgggaaccggaaaggcgggccagcagcctgcaagaaaaagattgaattttggtcagactggagacgcagactcagtacctgacccccagcctctcggacagccaccagcagccccctctggtctgggaactaatacgatggctacaggcagtggcgcaccaatggcagacaataacgagggcgccgacggagtgggtaattcctcgggaaattggcattgcgattccacatggatgggcgacagagtcatcaccaccagcacccgaacctgggccctgcccacctacaacaaccacctctacaaacaaatttccagccaatcaggagcctcgaacgacaatcactactttggctacagcaccccttgggggtattttgacttcaacagattccactgccacttttcaccacgtgactggcaaagactcatcaacaacaactggggattccgacccaagagactcaacttcaagctctttaacattcaagtcaaagaggtcacgcagaatgacggtacgacgacgattgccaataaccttaccagcacggttcaggtgtttactgactcggagtaccagctcccgtacgtcctcggctcggcgcatcaaggatgcctcccgccgttcccagcagacgtcttcatggtgccacagtatggatacctcaccctgaacaacgggagtcaggcagtaggacgctcttcattttactgcctggagtactttccttctcagatgctgcgtaccggaaacagctttaccttcagctacacttttgaggacgttcctttccacagcagctacgctcacagccagagtctggaccgtctcatgaatcctctcatcgaccagtacctgtattacttgagcagaacaaacactccaagtggaaccaccacgcagtcaaggcttcagttttctcaggccggagcgagtgacattcgggaccagtctaggaactggcttcctggaccctgttaccgccagcagcgagtatcaaagacatctgcggataacaacaacagtgaatactcgtggactggagctaccaagtaccacctcaatggcagagactctctggtgaatccgggcccggccatggcaagccacaaggacgatgaagaaaagttttttcctcagagcggggttctcatctttgggaagcaaggctcagagaaaacaaatgtggacattgaaaaggtcatgattacagacgaagaggaaatcaggacaaccaatcccgtggctacggagcagtatggttctgtatctaccaacctccagagaggcaacctagcagaccaagactacacaaaaactgctaggcaagcagctaccgcagatgtcaacacacaaggcgttcttccaggcatggtctggcaggacagagatgtgtaccttcaggggcccatctgggcaaagattccacacacggacggacattttcacccctctcccctcatgggtggattcggacttaaacaccctcctccccagattctcatcaagaacaccccggtacctgcgaatccttcgaccaccttcagtgcggcaaagtttgcttccttcatcacacagtactccacgggacaggtcagcgtggagatcgagtgggagctgcagaaggaaaacagcaaacgctggaatcccgaaattcagtacacttccaactacaacaagtctattaatgtggactttactgtggacactaatggcgtgtattcagagcctcgccccattggcaccagatacctgactcgtaatctgtaa

SEQ ID NO: 60 - protein, 745 aa, synthetic construct
  REGION 1..745: note = synthetically generated sequence
MAADGYLPDWLEDTLSEGIRQWWKLKPGPPPPKPAERHKDDSRGLVLPGYKYLGPFNGLDKGEPVNAADAAALEHDKAYDRQLDSGDNPYLKYNHADAEFQERLKEDTSFGGNLGRAVFQAKKRVLEPLGLVEEPVKTAPGKKRPVEHSPVEPDSSSGTGKAGQQPARKRLNFGQTGDADSVPDPQPLGQPPAAPSGLGTNTMATGSGAPMADNNEGADGVGNSSGNWHCDSTWMGDRVITTSTRTWALPTYNNHLYKQISSQSGASNDNHYFGYSTPWGYFDFNRFHCHFSPRDWQRLINNNWGFRPKRLNFKLFNIQVKEVTQNDGTTTIANNLTSTVQVFTDSEYQLPYVLGSAHQGCLPPFPADVFMVPQYGYLTLNNGSQAVGRSSFYCLEYFPSQMLRTGNSFTFSYTFEDVPFHSSYAHSQSLDRLMNPLIDQYLYYLSRTNTPSGTTTQSRLQFSQAGASDIRDQSRNWLPGPCYRQQRVSKTSADNNNSEYSWTGATKYHLNGRDSLVNPGPAMASHKDDEEKFFPQSGVLIFGKQGSEKTNVDIEKVMITDEEEIRTTNPVATEQYGSVSTNLQRGNLADQDYTKTARQAATADVNTQGVLPGMVWQDRDVYLQGPIWAKIPHTDGHFHPSPLMGGFGLKHPPPQILIKNTPVPANPSTTFSAAKFASFITQYSTGQVSVEIEWELQKENSKRWNPEIQYTSNYNKSINVDFTVDTNGVYSEPRPIGTRYLTRNL

SEQ ID NO: 61 - DNA, 2238 bp, synthetic construct; identical to SEQ ID NO: 3
  misc_feature 1..2238: note = synthetically generated sequence
  source 1..2238: mol_type = other DNA

SEQ ID NO: 62 - protein, 745 aa, synthetic construct; identical to SEQ ID NO: 16
  REGION 1..745: note = synthetically generated sequence

SEQ ID NO: 63 - DNA, 2238 bp, synthetic construct
  misc_feature 1..2238: note = synthetically generated sequence
  source 1..2238: mol_type = other DNA
atggctgccgatggttatcttccagattggctcgaggacactctctctgaaggaataagacagtggtggaagctcaaacctggcccaccaccaccaaagcccgcagagcggcttaaggacgacagcaggggtcttgtgcttcctgggtacaagtacctcggacccttcaacggactcgacaagggagagccggtcaacgccgcagacgccgcggccctcgagcacgacaaagcctacgaccggcagctcgacagcggagacaacccgtacctcaagtacaaccacgccgacgcggagtttcaggagcgccttaaagaagatacgtcttttgggggcaacctcggacgagcagtcttccaggcgaaaaagagggttcttgaacctctgggcctggttgaggaacctgttaagacggctccgggaaaaaagaggccggtagcccactctcctgtggagccagactcctcctcgggaaccggaaaggcgggccagcagcctgcaagaaaaagattgaattttggtcagactggagacgcagactcagtacctgacccccagcctctcggacagccaccagcagccccctctggtctgggaactaatacgatggctacaggcggtggcgcaccaatggcagacaataacgagggcgccgacggagtgggtaattcctcgggaaattggcattgcgattccacatggatgggcgacagagtcatcaccaccagcacccgaacctgggccctgcccacctacaacaaccacctctacaaacaaatttccagccaatcaggagcctcgaacgacaatcactactttggctacagcaccccttgggggtattttgacttcaacagattccactgccacttttcaccacgtgactggcaaagactcatcaacaacaactggggattccgacccaagagactcaacttcaagctctttaacattcaagtcaaagaggtcacgcagaatgacggtacgacgacgattgccaataaccttaccagcacggttcaggtgtttactgactcggagtaccagctcccgtacgtcctcggctcggcgcatcaaggatgcctcccgccgttcccagcagacgtcttcatggtgccacagtatggatacctcaccctgaacaacgggagtcaggcagtaggacgctcttcattttactgcctggagtactttccttctcagatgctgcgtaccggaaacagctttaccttcagctacacttttgaggacgttcctttccacagcagctacgctcacagccagagtctggaccgtctcatgaatcctctcatcgaccagtacctgtattacttgagcagaacaaacactccaagtggaaccaccacgcagtcaaggcttcagttttctcaggccggagcgagtgacattcgggaccagtctaggaactggcttcctggaccctgttaccgccagcagcgagtatcaaagacatctgcggataacaacaacagtgaatactcgtggactggagctaccaagtaccacctcaatggcagagactctctggtgaatccgggcccggccatggcaagccacaaggacgatgaagaaaagttttttcctcagagcggggttctcatctttgggaagcaaggctcagagaaaacaaatgtggacattgaaaaggtcatgattacagacgaagaggaaatcaggacaaccaatcccgtggctacggagcagtatggttctgtatctaccaacctccagagaggcaacctagcacacgacatcaccaagaatattgctaggcaagcagctaccgcagatgtcaacacacaaggcgttcttccaggcatggtctggcaggacagagatgtgtaccttcaggggcccatctgggcaaagattccacacacggacggacattttcacccctctcccctcatgggtggattcggacttaaacaccctcctccccagattctcatcaagaacaccccggtacctgcgaatccttcgaccaccttcagtgcggcaaagtttgcttccttcatcacacagtactccacgggacaggtcagcgtggagatcgagtgggagctgcagaaggaaaacagcaaacgctggaatcccgaaattcagtacacttccaactacaacaagtctattaatgtggactttactgtggacactaatggcgtgtattcagagcctcgccccattggcaccagatacctgactcgtaatctgtaa

SEQ ID NO: 64 - protein, 745 aa, synthetic construct
  REGION 1..745: note = synthetically generated sequence
MAADGYLPDWLEDTLSEGIRQWWKLKPGPPPPKPAERLKDDSRGLVLPGYKYLGPFNGLDKGEPVNAADAAALEHDKAYDRQLDSGDNPYLKYNHADAEFQERLKEDTSFGGNLGRAVFQAKKRVLEPLGLVEEPVKTAPGKKRPVAHSPVEPDSSSGTGKAGQQPARKRLNFGQTGDADSVPDPQPLGQPPAAPSGLGTNTMATGGGAPMADNNEGADGVGNSSGNWHCDSTWMGDRVITTSTRTWALPTYNNHLYKQISSQSGASNDNHYFGYSTPWGYFDFNRFHCHFSPRDWQRLINNNWGFRPKRLNFKLFNIQVKEVTQNDGTTTIANNLTSTVQVFTDSEYQLPYVLGSAHQGCLPPFPADVFMVPQYGYLTLNNGSQAVGRSSFYCLEYFPSQMLRTGNSFTFSYTFEDVPFHSSYAHSQSLDRLMNPLIDQYLYYLSRTNTPSGTTTQSRLQFSQAGASDIRDQSRNWLPGPCYRQQRVSKTSADNNNSEYSWTGATKYHLNGRDSLVNPGPAMASHKDDEEKFFPQSGVLIFGKQGSEKTNVDIEKVMITDEEEIRTTNPVATEQYGSVSTNLQRGNLAHDITKNIARQAATADVNTQGVLPGMVWQDRDVYLQGPIWAKIPHTDGHFHPSPLMGGFGLKHPPPQILIKNTPVPANPSTTFSAAKFASFITQYSTGQVSVEIEWELQKENSKRWNPEIQYTSNYNKSINVDFTVDTNGVYSEPRPIGTRYLTRNL

SEQ ID NO: 65 - DNA, 2238 bp, synthetic construct
  misc_feature 1..2238: note = synthetically generated sequence
  source 1..2238: mol_type = other DNA
atggctgccgatggttatcttccagattggctcgaggacactctctctgaaggaataagacagtggtggaagctcaaacctggcccaccaccaccaaagcccgcagggcggcataaggacgacagcaggggtcttgtgcttcctgggtacaagtacctcggacccttcaacggactcgacaagggagagccggtcaacgaggcagacgccgcggccctcgagcacgacaaagcctacgaccggcagctcgacagcggagacaacccgtacctcaagtacaaccacgccgacgcggagtttcaggagcgccttaaagaagatacgtcttttgggggcaacctcggacgagcagtcttccaggcgaaaaagagggttcttgaacctctgggcctggttgaggaacctgttaagacggctccgggaaaaaagaggccggtagagcactctcctgtggagccagactcctcctcgggaaccggaaaggcgggccagcagcctgcaagaaaaagattgaattttggtcagactggagacgcagactcagtacctgacccccagcctctcggacagccaccagcagccccctctggtctgggaactaatacgatggctacaggcagtggcgcaccaatggcagacaataacgagggcgccgacggagtgggtaattcctcgggagattggcattgcgattccacatggatgggcgacagagtcatcaccaccagcacccgaacctgggccctgcccacctacaacaaccacctctacaaacaaatttccagccaatcaggagcctcgaacgacaatcactactttggctacagcaccccttgggggtattttgacttcaacagattccactgccacttttcaccacgtgactggcaaagactcatcaacaacaactggggattccgacccaagagactcaacttcaagctctttaacattcaagtcaaagaggtcacgcagaatgacggtacgacgacgattgccaataaccttaccagcacggttcaggtgtttactgactcggagtaccagctcccgtacgtcctcggctcggcgcatcaaggatgcctcccgccgttcccagcagacgtcttcatggtgccacagtatggatacctcaccctgaacaacgggagtcaggcagtaggacgctcttcattttactgcctggagtactttccttctcagatgctgcgtaccggaaacaactttaccttcagctacacttttgaggacgttcctttccacagcagctacgctcacagccagagtctggaccgtctcatgaatcctctcatcgaccagtacctgtattacttgagcagaacaaacactccaagtggaaccaccacgcagtcaaggcttcagttttctcaggccggagcgagtgacattcgggaccagtctaggaactggcttcctggaccctgttaccgccagcagcgagtatcaaagacacctgcggataacaacaacagtgaatactcgtggactggagctaccaagtaccacctcaatggcagagactctctggtgaatccgggcccggccatggcaagccacaaggacgatgaagaaaagttttttcctcagagcggggttctcatctttgggaagcaaggctcagagaaaacaaatgtggacattgaaaaggtcatgattacagacgaagaggaaatcaggacaaccaatcccgtggctacggagcagtatggttctgtatctaccaacctccagagaggcagcctagcaaaccaagactacacaaaaactgctaggcaagcagctaccgcagatgtcaacacacaaggcgttcttccaggcatggtctggcaggacagagatgtgtaccttcaggggcccatctgggcaaagattccacacacggacggacattttcacccctctcccctcatgggtggattcggacttaaacaccctcctccccagattctcatcaagaacaccccggtacctgcgaatccttcgaccaccttcagtgcggcaaagtttgcttccttcatcacacagtactccacgggacaggtcagcgtggagatcgagtgggagctgcagaaggaaaacagcaaacgctggaatcccgaaattcagtacacttccaactacaacaagtctattaatgtggactttactgtggacactaatggcgtgtattcagagcctcgccccattggcaccagatacctgactcgtaatctgtaa

SEQ ID NO: 66 - protein, 745 aa, synthetic construct
  REGION 1..745: note = synthetically generated sequence
MAADGYLPDWLEDTLSEGIRQWWKLKPGPPPPKPAGRHKDDSRGLVLPGYKYLGPFNGLDKGEPVNEADAAALEHDKAYDRQLDSGDNPYLKYNHADAEFQERLKEDTSFGGNLGRAVFQAKKRVLEPLGLVEEPVKTAPGKKRPVEHSPVEPDSSSGTGKAGQQPARKRLNFGQTGDADSVPDPQPLGQPPAAPSGLGTNTMATGSGAPMADNNEGADGVGNSSGDWHCDSTWMGDRVITTSTRTWALPTYNNHLYKQISSQSGASNDNHYFGYSTPWGYFDFNRFHCHFSPRDWQRLINNNWGFRPKRLNFKLFNIQVKEVTQNDGTTTIANNLTSTVQVFTDSEYQLPYVLGSAHQGCLPPFPADVFMVPQYGYLTLNNGSQAVGRSSFYCLEYFPSQMLRTGNNFTFSYTFEDVPFHSSYAHSQSLDRLMNPLIDQYLYYLSRTNTPSGTTTQSRLQFSQAGASDIRDQSRNWLPGPCYRQQRVSKTPADNNNSEYSWTGATKYHLNGRDSLVNPGPAMASHKDDEEKFFPQSGVLIFGKQGSEKTNVDIEKVMITDEEEIRTTNPVATEQYGSVSTNLQRGSLANQDYTKTARQAATADVNTQGVLPGMVWQDRDVYLQGPIWAKIPHTDGHFHPSPLMGGFGLKHPPPQILIKNTPVPANPSTTFSAAKFASFITQYSTGQVSVEIEWELQKENSKRWNPEIQYTSNYNKSINVDFTVDTNGVYSEPRPIGTRYLTRNL

SEQ ID NO: 67 - DNA, 2238 bp, synthetic construct
  misc_feature 1..2238: note = synthetically generated sequence
  source 1..2238: mol_type = other DNA
atggctgccgatggttatcttccagattggctcgaggacactctctctgaaggaataagacagtggtggaagctcaaacctggcccaccaccaccaaagcccgcagggcggcataaggacgacagcaggggtcttgtgcttcctgggtacaagtacctcggacccttcaacggactcgacaagggagagccggtcaacgccgcagacgccgcggccctcgagcacgacaaagcctacgaccggcagctcgacagcggagacaacccgtacctcaagtacaaccacgccgacgcggagtttcaggagcgccttaaagaagatacgtcttttgggggcaacctcggacgagcagtcttccaggcgaaaaagagggttcttgaacctctgggcctggttgaggaacctgttaagacggctccgggaaaaaagaggccggtagagcactctcctgtggagccagactcctcctcgggaaccggaaaggcgggccagcagcctgcaagaaaaagattgaattttggtcagactggagacgcagactcagtacctgacccccagcctctcggacagccaccagcagccccctctggtctgggaactaatacgatggctacaggcagtggcgcaccaatggcagacaataacgagggcgccgacggagtgggtaattcctcgggaaattggcattgcgattccacatggatgggcgacagagtcatcaccaccagcacccgaacctgggccctgcccacctacaacaaccacctctacaaacaaatttccagccaatcaggagcctcgaacgacaatcactactttggctacagcaccccttgggggtattttgacttcaacagattccactgccacttttcaccacgtgactggcaaagactcatcaacaacaactggggattccgacccaagagactcaacttcaagctctttaacattcaagtcaaagaggtcacgcagaatgacggtacgacgacgattgccaataaccttaccagcacggttcaggtgtttactgactcggagtaccagctcccgtacgtcctcggctcggcgcatcaaggatgcctcccgccgttcccagcagacgtcttcatggtgccacagtatggatacctcaccctgaacaacgggagtcaggcagtaggacgctcttcattttactgcctggagtactttccttctcagatgctgcgtaccggaaacagctttaccttcagctacacttttgaggacgttcctttccacagcagctacgctcacagccagagtctggaccgtctcatgaatcctctcatcgaccagtacctgtattacttgagcagaacaaacactccaagtggaaccaccacgcagtcaaggcttcagttttctcaggccggagcgagtgacattcgggaccagtctaggaactggcttcctggaccctgttaccgccagcagcgagtatcaaagacatctgcggataacaacaacagtgaatactcgtggactggagctaccaagtaccacctcaatggcagagactctctggtgaatccgggcccggccatggcaagccacaaggacgatgaagaaaagttttttcctcagagcggggttctcatctttgggaagcaaggctcagagaaaacaaatgtggacattgaaaaggtcatgattacagacgaagaggaaatcaggacaaccaatcccgtggctacggagcagtatggttctgtatctaccaacctccagagaggcaacctagcacacgacatcaccaagaatattgctaggcaagcagctaccgcagatgtcaacacacaaggcgttcttccaggcatggtctggcaggacagagatgtgtaccttcaggggcccatctgggcaaagattccacacacggacggacattttcacccctctcccctcatgggtggattcggacttaaacaccctcctccccagattctcatcaagaacaccccggtacctgcgaatccttcgaccaccttcagtgcggcaaagtttgcttccttcatcacacagtactccacgggacaggtcagcgtggagatcgagtgggagctgcagaaggaaaacagcaaacgctggaatcccgaaattcagtacacttccaactacaacaagtctattaatgtggactttactgtggacactaatggcgtgtattcagagcctcgccccattggcaccagatacctgactcgtaatctgtaa

SEQ ID NO: 68 - protein, 745 aa, synthetic construct
  REGION 1..745: note = synthetically generated sequence
MAADGYLPDWLEDTLSEGIRQWWKLKPGPPPPKPAGRHKDDSRGLVLPGYKYLGPFNGLDKGEPVNAADAAALEHDKAYDRQLDSGDNPYLKYNHADAEFQERLKEDTSFGGNLGRAVFQAKKRVLEPLGLVEEPVKTAPGKKRPVEHSPVEPDSSSGTGKAGQQPARKRLNFGQTGDADSVPDPQPLGQPPAAPSGLGTNTMATGSGAPMADNNEGADGVGNSSGNWHCDSTWMGDRVITTSTRTWALPTYNNHLYKQISSQSGASNDNHYFGYSTPWGYFDFNRFHCHFSPRDWQRLINNNWGFRPKRLNFKLFNIQVKEVTQNDGTTTIANNLTSTVQVFTDSEYQLPYVLGSAHQGCLPPFPADVFMVPQYGYLTLNNGSQAVGRSSFYCLEYFPSQMLRTGNSFTFSYTFEDVPFHSSYAHSQSLDRLMNPLIDQYLYYLSRTNTPSGTTTQSRLQFSQAGASDIRDQSRNWLPGPCYRQQRVSKTSADNNNSEYSWTGATKYHLNGRDSLVNPGPAMASHKDDEEKFFPQSGVLIFGKQGSEKTNVDIEKVMITDEEEIRTTNPVATEQYGSVSTNLQRGNLAHDITKNIARQAATADVNTQGVLPGMVWQDRDVYLQGPIWAKIPHTDGHFHPSPLMGGFGLKHPPPQILIKNTPVPANPSTTFSAAKFASFITQYSTGQVSVEIEWELQKENSKRWNPEIQYTSNYNKSINVDFTVDTNGVYSEPRPIGTRYLTRNL

SEQ ID NO: 69 - DNA, 2238 bp, synthetic construct
  misc_feature 1..2238: note = synthetically generated sequence
  source 1..2238: mol_type = other DNA
atggctgccgatggttatcttccagattggctcgaggacactctctctgaaggaataagacagtggtggaagctcaaacctggcccaccaccaccaaagcccgcagagcggcataaggacggcagcaggggtcttgtgcttcctgggtacaagtacctcggacccttcaacggactcgacaagggagagccggtcaacgccgcagacgccgcggccctcgagcacgacaaagcctacgaccggcagctcgacagcggagacaacccgtacctcaagtacaaccacgccgacgcggagtttcaggagcgccttgaagaagatacgtcttttgggggcaacctcggacgagcagtcttccaggcgaaaaagagggttcttgaacctctgggcctggttgaggaacctgttaagacggctccgggaaaaaagaggccggtagagcactctcctgtggagccagactcctcctcgggaaccggaaaggcggaccagcagcctgcaagaaaaagattgaattttggtcagactggagacgcagactcagtacctgacccccagcctctcggacagccaccagcagccccctctggtctgggaactaatacgatggctacaggcagtggcgcaccaatggcagacaataacgagggcgccgacggagtgggtaattcctcgggaaattggcattgcgattccacatggatgggcgacagagtcatcaccaccagcacccgaacctgggccctgcccacctacaacaaccacctctacaaacaaatttccagccaatcaggagcctcgaacgacaatcactactttggctacagcaccccttgggggtattttgacttcaacagattccactgccacttttcaccacgtgactggcaaagactcatcaacaacaactggggattccgacccaagagactcaacttcaagctctttaacattcaagtcaaagaggtcacgcagaatgacggtacgacgacgattgccaataaccttaccagcacggttcaggtgtttactgactcggagtaccagctcccgtacgtcctcggctcggcgcatcaaggatgcctcccgccgttcccagcagacgtcttcatggtgccacagtatggatacctcaccctgaacaacgggagtcaggcagtaggacgctcttcattttactgcctggagtactttccttctcagatgctgcgtaccggaaacaactttaccttcagctacacttttgaggacgttcctttccacagcagctacgctcacagccagagtctggaccgtctcatgaatcctctcatcgaccagtacctgtattacttgagcagaacaaacactccaagtggaaccaccacgcagtcaaggcttcagttttctcaggccggagcgagtgacattcgggaccagtctaggaactggcttcctggaccctgttaccgccagcagcgagtatcaaagacacctgcggataacaacaacagtgaatactcgtggactggagctaccaagtaccacctcaatggcagagactctctggtgaatccgggcccggccatggcaagccacaaggacgatgaagaaaagttttttcctcagagcggggttctcatctttgggaagcaaggctcagagaaaacaaatgtggacattgaaaaggtcatgattacagacgaagaggaaatcaggacaaccaatcccgtggctacggagcagtatggttctgtatctaccaacctccagagaggcaacctagcaaaccaagactacacaaaaactgctaggcaagcagctaccgcagatgtcaacacacaaggcgttcttccaggcatggtctggcaggacagagatgtgtaccttcaggggcccatctgggcaaagattccacacacggacggacattttcacccctctcccctcatgggtggattcggacttaaacaccctcctccccagattctcatcaagaacaccccggtacctgcgaatccttcgaccaccttcagtgcggcaaagtttgcttccttcatcacacagtactccacgggacaggtcagcgtggagatcgagtgggagctgcagaaggaaaacagcaaacgctggaatcccgaaattcagtacacttccaactacaacaagtctattaatgtggactttactgtggacactaatggcgtgtattcagagcctcgccccattggcaccagatacctgactcgtaatctgtaa

SEQ ID NO: 70 - protein, 745 aa, synthetic construct
  REGION 1..745: note = synthetically generated sequence
MAADGYLPDWLEDTLSEGIRQWWKLKPGPPPPKPAERHKDGSRGLVLPGYKYLGPFNGLDKGEPVNAADAAALEHDKAYDRQLDSGDNPYLKYNHADAEFQERLEEDTSFGGNLGRAVFQAKKRVLEPLGLVEEPVKTAPGKKRPVEHSPVEPDSSSGTGKADQQPARKRLNFGQTGDADSVPDPQPLGQPPAAPSGLGTNTMATGSGAPMADNNEGADGVGNSSGNWHCDSTWMGDRVITTSTRTWALPTYNNHLYKQISSQSGASNDNHYFGYSTPWGYFDFNRFHCHFSPRDWQRLINNNWGFRPKRLNFKLFNIQVKEVTQNDGTTTIANNLTSTVQVFTDSEYQLPYVLGSAHQGCLPPFPADVFMVPQYGYLTLNNGSQAVGRSSFYCLEYFPSQMLRTGNNFTFSYTFEDVPFHSSYAHSQSLDRLMNPLIDQYLYYLSRTNTPSGTTTQSRLQFSQAGASDIRDQSRNWLPGPCYRQQRVSKTPADNNNSEYSWTGATKYHLNGRDSLVNPGPAMASHKDDEEKFFPQSGVLIFGKQGSEKTNVDIEKVMITDEEEIRTTNPVATEQYGSVSTNLQRGNLANQDYTKTARQAATADVNTQGVLPGMVWQDRDVYLQGPIWAKIPHTDGHFHPSPLMGGFGLKHPPPQILIKNTPVPANPSTTFSAAKFASFITQYSTGQVSVEIEWELQKENSKRWNPEIQYTSNYNKSINVDFTVDTNGVYSEPRPIGTRYLTRNL

SEQ ID NO: 71 - DNA, 2238 bp, synthetic construct
  misc_feature 1..2238: note = synthetically generated sequence
  source 1..2238: mol_type = other DNA
atggctgccgatggttatcttccagattggctcgaggacactctctctgaaggaataagacagtggtggaagctcaaacctggcccaccaccaccaaagcccgcagagcggcataaggacgacagcaggggtcttgtgcttcctgggtacaagtacctcggacccttcaacggactcgacaagggagagccggtcaacgaggcagacgccgcggccctcgagcacgacaaagcctacgaccggcagctcgacagcggagacaacccgtacctcaagtacaaccacgccgacgcggagtttcaggagcgccttaaagaagatacgtcttttgggggcaacctcggacgagcagtcttccaggcgaaaaagagggttcttgaacctctgggcctggttgaggaacctgttaagacggctccgggaaaaaagaggccggtagagcactctcctgtggagccagactcctcctcgggaaccggaaaggcgggccagcagcctgcaagaaaaagattgaattttggtcagactggagacgcagactcagtacctgacccccagcctctcggacagccaccagcagccccctctggtctgggaactaatacgatggctacaggcagtggcgcaccaatggcagacaataacgagggcgccgacggagtgggtaattcctcgggaaattggcattgcgattccacatggatgggcgacagagtcatcaccaccagcacccgaacctgggccctgcccacctacaacaaccacctctacaaacaaatttccagccaatcaggagcctcgaacgacaatcactactttggctacagcaccccttgggggtattttgacttcaacagattccactgccacttttcaccacgtgactggcaaagactcatcaacaacaactggggattccgacccaagagactcaacttcaagctctttaacattcaagtcaaagaggtcacgcagaatgacggtacgacgacgattgccaataaccttaccagcacggttcaggtgtttactgactcggagtaccagctcccgtacgtcctcggctcggcgcatcaaggatgcctcccgccgttcccagcagacgtcttcatggtgccacagtatggatacctcaccctgaacaacgggagtcaggcagtaggacgctcttcattttactgcctggagtactttccttctcagatgctgcgtaccggaaacaactttaccttcagctacacttttgaggacgttcctttccacagcagctacgctcacagccagagtctggaccgtctcatgaatcctctcatcgaccagtacctgtattacttgagcagaacaaacactccaagtggaaccaccacgcagtcaaggcttcagttttctcaggccggagcgagtgacattcgggaccagtctaggaactggcttcctggaccctgttaccgccagcagcgagtatcaaagacatctgcggataacaacaacagtgaatactcgtggactggagctaccaagtaccacctcaatggcagagactctctggtgaatccgggcccggccatggcaagccacaaggacgatgaagaaaagttttttcctcagagcggggttctcatctttgggaagcaaggctcagagaaaacaaatgtggacattgaaaaggtcatgattacagacgaagaggaaatcagggcaaccaatcccgtggctacggagcagtatggttctgtatctaccaacctccagagaggcaacctagcagaccaagactacacaaaaactgctaggcaagcagctaccgcagatgtcaacacacaaggcgttcttccaggcatggtctggcaggacagagatgtgtaccttcaggggcccatctgggcaaagattccacacacggacggacattttcacccctctcccctcatgggtggattcggacttaaacaccctcctccccagattctcatcaagaacaccccggtacctgcgaatccttcgaccaccttcagtgcggcaaagtttgcttccttcatcacacagtactccacgggacaggtcagcgtggagatcgagtgggagctgcagaaggaaaacagcaaacgctggaatcccgaaattcagtacacttccaactacaacaagtctattaatgtggactttactgtggacactaatggcgtgtattcagagcctcgccccattggcaccagatacctgactcgtaatctgtaa

SEQ ID NO: 72 - protein, 745 aa, synthetic construct
  REGION 1..745: note = synthetically generated sequence
MAADGYLPDWLEDTLSEGIRQWWKLKPGPPPPKPAERHKDDSRGLVLPGYKYLGPFNGLDKGEPVNEADAAALEHDKAYDRQLDSGDNPYLKYNHADAEFQERLKEDTSFGGNLGRAVFQAKKRVLEPLGLVEEPVKTAPGKKRPVEHSPVEPDSSSGTGKAGQQPARKRLNFGQTGDADSVPDPQPLGQPPAAPSGLGTNTMATGSGAPMADNNEGADGVGNSSGNWHCDSTWMGDRVITTSTRTWALPTYNNHLYKQISSQSGASNDNHYFGYSTPWGYFDFNRFHCHFSPRDWQRLINNNWGFRPKRLNFKLFNIQVKEVTQNDGTTTIANNLTSTVQVFTDSEYQLPYVLGSAHQGCLPPFPADVFMVPQYGYLTLNNGSQAVGRSSFYCLEYFPSQMLRTGNNFTFSYTFEDVPFHSSYAHSQSLDRLMNPLIDQYLYYLSRTNTPSGTTTQSRLQFSQAGASDIRDQSRNWLPGPCYRQQRVSKTSADNNNSEYSWTGATKYHLNGRDSLVNPGPAMASHKDDEEKFFPQSGVLIFGKQGSEKTNVDIEKVMITDEEEIRATNPVATEQYGSVSTNLQRGNLADQDYTKTARQAATADVNTQGVLPGMVWQDRDVYLQGPIWAKIPHTDGHFHPSPLMGGFGLKHPPPQILIKNTPVPANPSTTFSAAKFASFITQYSTGQVSVEIEWELQKENSKRWNPEIQYTSNYNKSINVDFTVDTNGVYSEPRPIGTRYLTRNL

SEQ ID NO: 73 - DNA, 2238 bp, synthetic construct
  misc_feature 1..2238: note = synthetically generated sequence
  source 1..2238: mol_type = other DNA
atggctgccgatggttatcttccagattggctcgaggacactctctctgaaggaataagacagtggtggaagctcaaacctggcgcaccaccaccaaagcccgcagagcggcataaggacgacagcaggggtcttgtgcttcctgggtacaagtacctcggacccttcaacggactcgacaagggagagccggtcaacgccgcagacgccgcggccctcgagcacgacaaagcctacgaccggcagctcgacagcggagacaacccgtacctcaagtacaaccacgccgacgcggagtttcaggagcgccttgaagaagatacgtcttttgggggcaacctcggacgagcagtcttccaggcgaaaaagagggttcttgaacctctgggcctggttgaggaacctgttaagacggctccgggaaaaaagaggccggtagagcactctcctgtggagccagactcctcctcgggaaccggaaaggcgggccagcagcctgcaagaaaaagattgaattttggtcagactggagacgcagactcagtacctgacccccagcctctcggacagccaccagcagccccctctggtctgggaactaatacgatggctacaggcggtggcgcaccaatggcagacaataacgagggcgccgacggagtgggtaattcctcgggaaattggcattgcgattccacatggatgggcgacagagtcatcaccaccagcacccgaacctgggccctgcccacctacaacaaccacctctacaaacaaatttccagccaatcaggagcctcgaacgacaatcactactttggctacagcaccccttgggggtattttgacttcaacagattccactgccacttttcaccacgtgactggcaaagactcatcaacaacaactggggattccgacccaagagactcaacttcaagctctttaacattcaagtcaaagaggtcacgcagaatgacggtacgacgacgattgccaataaccttaccagcacggttcaggtgtttactgactcggagtaccagctcccgtacgtcctcggctcggcgcatcaaggatgcctcccgccgttcccagcagacgtcttcatggtgccacagtatggatacctcaccctgaacaacgggagtcaggcagtaggacgctcttcattttactgcctggagtactttccttctcagatgctgcgtaccggaaacaactttaccttcagctacacttttgaggacgttcctttccacagcagctacgctcacagccagagtctggaccgtctcatgaatcctctcatcgaccagtacctgtattacttgagcagaacaaacactccaagtggaaccaccacgcagtcaaggcttcagttttctcaggccggagcgagtgacattcgggaccagtctaggaactggcttcctggaccctgttaccgccagcagcgagtatcaaagacatctgcggataacaacaacagtgaatactcgtggactggagctaccaagtaccacctcaatggcagagactctctggtgaatccgggcccggccatggcaagccacaaggacgatgaagaaaagttttttcctcagagcggggttctcatctttgggaagcaaggctcagagaaaacaaatgtggacattgaaaaggtcatgattacagacgaagaggaaatcaggacaaccaatcccgtggctacggagcagtatggttctgtatctaccaacctccagagaggcaacctagcacagcctgacgccacaaaaaacgctaggcaagcagctaccgcagatgtcaacacacaaggcgttcttccaggcatggtctggcaggacagagatgtgtaccttcaggggcccatctgggcaaagattccacacacggacggacattttcacccctctcccctcatgggtggattcggacttaaacaccctcctccccagattctcatcaagaacaccccggtacctgcgaatccttcgaccaccttcagtgcggcaaagtttgcttccttcatcacacagtactccacgggacaggtcagcgtggagatcgagtgggagctgcagaaggaaaacagcaaacgctggaatcccgaaattcagtacacttccaactacaacaagtctattaatgtggactttactgtggacactaatggcgtgtattcagagcctcgccccattggcaccagatacctgactcgtaatctgtaa

SEQ ID NO: 74 - protein, 745 aa, synthetic construct
  REGION 1..745: note = synthetically generated sequence
MAADGYLPDWLEDTLSEGIRQWWKLKPGAPPPKPAERHKDDSRGLVLPGYKYLGPFNGLDKGEPVNAADAAALEHDKAYDRQLDSGDNPYLKYNHADAEFQERLEEDTSFGGNLGRAVFQAKKRVLEPLGLVEEPVKTAPGKKRPVEHSPVEPDSSSGTGKAGQQPARKRLNFGQTGDADSVPDPQPLGQPPAAPSGLGTNTMATGGGAPMADNNEGADGVGNSSGNWHCDSTWMGDRVITTSTRTWALPTYNNHLYKQISSQSGASNDNHYFGYSTPWGYFDFNRFHCHFSPRDWQRLINNNWGFRPKRLNFKLFNIQVKEVTQNDGTTTIANNLTSTVQVFTDSEYQLPYVLGSAHQGCLPPFPADVFMVPQYGYLTLNNGSQAVGRSSFYCLEYFPSQMLRTGNNFTFSYTFEDVPFHSSYAHSQSLDRLMNPLIDQYLYYLSRTNTPSGTTTQSRLQFSQAGASDIRDQSRNWLPGPCYRQQRVSKTSADNNNSEYSWTGATKYHLNGRDSLVNPGPAMASHKDDEEKFFPQSGVLIFGKQGSEKTNVDIEKVMITDEEEIRTTNPVATEQYGSVSTNLQRGNLAQPDATKNARQAATADVNTQGVLPGMVWQDRDVYLQGPIWAKIPHTDGHFHPSPLMGGFGLKHPPPQILIKNTPVPANPSTTFSAAKFASFITQYSTGQVSVEIEWELQKENSKRWNPEIQYTSNYNKSINVDFTVDTNGVYSEPRPIGTRYLTRNL

SEQ ID NO: 75 - DNA, 2238 bp, synthetic construct
  misc_feature 1..2238: note = synthetically generated sequence
  source 1..2238: mol_type = other DNA
atggctgccgatggttatcttccagattggctcgaggacactctctctgaaggaataagacagtggtggaagctcaaacctggcccaccaccaccaaagcccgcagagcggcataaggacgacagcaggggtcttgtgcttcctgggtacaagtacctcggacccttcaacggactcgacaagggagagccggtcaacgaggcagacgccgcggccctcgagcacgacaaagcctacgaccggcagctcgacagcggagacaacccgtacctcaagtacaaccacgccgacgcggagtttcaggagcgccttaaagaagatacgtcttttgggggcaacctcggacgagcagtcttccaggcgaaaaagagggttcttgaacctctgggcctggttgaggaacctgttaagacggctccgggaaaaaagaggccggtagagcactctcctgtggagccagactcctcctcgggaaccggaaaggcgggccagcagcctgcaagaaaaagattgaattttggtcagactggagacgcagactcagtacctgacccccagcctctcggacagccaccagcagccccctctggtctgggaactaatacgatggctacaggcagtggcgcaccaatggcagacaataacgagggcgccgacggagtgggtaattcctcgggaaattggcattgcgattccacatggatgggcgacagagtcatcaccaccagcacccgaacctgggccctgcccacctacaacaaccacctctacaaacaaatttccagccaatcaggagcctcgaacgacaatcactactttggctacagcaccccttgggggtattttgacttcaacagattccactgccacttttcaccacgtgactggcaaagactcatcaacaacaactggggattccgacccaagagactcaacttcaagctctttaacattcaagtcaaagaggtcacgcagaatgacggtacgacgacgattgccaataaccttaccagcacggttcaggtgtttactgactcggagtaccagctcccgtacgtcctcggctcggcgcatcaaggatgcctcccgccgttcccagcagacgtcttcatggtgccacagtatggatacctcaccctgaacaacgggagtcaggcagtaggacgctcttcattttactgcctggagtactttccttctcagatgctgcgtaccggaaacaactttaccttcagctacacttttgaggacgttcctttccacagcagctacgctcacagccagagtctggaccgtctcatgaatcctctcatcgaccagtacctgtattacttgagcagaacaaacactccaagtggaaccaccacgcagtcaaggcttcagttttctcaggccggagcgagtgacattcgggaccagtctaggaactggcttcctggaccctgttaccgccagcagcgagtatcaaagacatctgcggataacaacaacagtgaatactcgtggactggagctaccaagtaccacctcaatggcagagactctctggtgaatccgggcccggccatggcaagccacaaggacgatgaagaaaagttttttcctcagagcggggttctcatctttgggaagcaaggctcagagaaaacaaatgtggacattgaaaaggtcatgattacagacgaagaggaaatcaggacaaccaatcccgtggctacggagcagtatggttctgtatctaccaacctccagagaggcaacctagcaaaggatcagacaaaaagcaccgctaggcaagcagctaccgcagatgtcaacacacaaggcgttcttccaggcatggtctggcaggacagagatgtgtaccttcaggggcccatctgggcaaagattccacacacggacggacattttcacccctctcccctcatgggtggattcggacttaaacaccctcctccccagattctcatcaagaacaccccggtacctgcgaatccttcgaccaccttcagtgcggcaaagtttgcttccttcatcacacagtactccacgggacaggtcagcgtggagatcgagtgggagctgcagaaggaaaacagcaaacgctggaatcccgaaattcagtacacttccaactacaacaagtctattaatgtggactttactgtggacactaatggcgtgtattcagagcctcgccccattggcaccagatacctgactcgtaatctgtaa

SEQ ID NO: 76 - protein, 745 aa, synthetic construct
  REGION 1..745: note = synthetically generated sequence
MAADGYLPDWLEDTLSEGIRQWWKLKPGPPPPKPAERHKDDSRGLVLPGYKYLGPFNGLDKGEPVNEADAAALEHDKAYDRQLDSGDNPYLKYNHADAEFQERLKEDTSFGGNLGRAVFQAKKRVLEPLGLVEEPVKTAPGKKRPVEHSPVEPDSSSGTGKAGQQPARKRLNFGQTGDADSVPDPQPLGQPPAAPSGLGTNTMATGSGAPMADNNEGADGVGNSSGNWHCDSTWMGDRVITTSTRTWALPTYNNHLYKQISSQSGASNDNHYFGYSTPWGYFDFNRFHCHFSPRDWQRLINNNWGFRPKRLNFKLFNIQVKEVTQNDGTTTIANNLTSTVQVFTDSEYQLPYVLGSAHQGCLPPFPADVFMVPQYGYLTLNNGSQAVGRSSFYCLEYFPSQMLRTGNNFTFSYTFEDVPFHSSYAHSQSLDRLMNPLIDQYLYYLSRTNTPSGTTTQSRLQFSQAGASDIRDQSRNWLPGPCYRQQRVSKTSADNNNSEYSWTGATKYHLNGRDSLVNPGPAMASHKDDEEKFFPQSGVLIFGKQGSEKTNVDIEKVMITDEEEIRTTNPVATEQYGSVSTNLQRGNLAKDQTKSTARQAATADVNTQGVLPGMVWQDRDVYLQGPIWAKIPHTDGHFHPSPLMGGFGLKHPPPQILIKNTPVPANPSTTFSAAKFASFITQYSTGQVSVEIEWELQKENSKRWNPEIQYTSNYNKSINVDFTVDTNGVYSEPRPIGTRYLTRNL

SEQ ID NO: 77 - DNA, 2238 bp, synthetic construct
  misc_feature 1..2238: note = synthetically generated sequence
  source 1..2238: mol_type = other DNA
atggctgccgatggttatcttccagattggctcgaggacactctctctgaaggaataagacagtggtggaagctcaaacctggcccaccaccaccaaagcccgcagagcggcataaggacgacagcaggggtcttgtgcttcctgggtacaagtacctcggacccttcaacggactcgacaagggagagccggtcaacgccgcagacgccgcggccctcgagcacgacaaagcctacgaccggcagctcgacagcggagacaacccgtacctcaagtacaaccacgccgacgcggagtttcaggagcgccttaaagaagatacgtcttttgggggcaacctcggacgagcagtcttccaggcgaaaaagagggttcttgaacctctgggcctggttgaggaacctgttaagacggctccgggaaaaaagaggccggtagagcactctcctgtggagccagactcctcctcgggaaccggaaaggcgggccagcagcctgcaagaaaaagattgaattttggtcagactggagacgcagactcagtacctgacccccagcctctcggacagccaccagcagccccctctggtctgggaactaatacgatggctacaggcggtggcgcaccaatggcagacaataacgagggcgccgacggagtgggtaattcctcgggaaattggcattgcgattccacatggatgggcgacagagtcatcaccaccagcacccgaacctgggccctgcccacctacaacaaccacctctacaaacaaatttccagccaatcaggagcctcgaacgacaatcactactttggctacagcaccccttgggggtattttgacttcaacagattccactgccacttttcaccacgtgactggcaaagactcatcaacaacaactggggattccgacccaagagactcaacttcaagctctttaacattcaagtcaaagaggtcacgcagaatgacggtacgacgacgattgccaataaccttaccagcacggttcaggtgtttactgactcggagtaccagctcccgtacgtcctcggctcggcgcatcaaggatgcctcccgccgttcccagcagacgtcttcatggtgccacagtatggatacctcaccctgaacaacgggagtcaggcagtaggacgctcttcattttactgcctggagtactttccttctcagatgctgcgtaccggaaacagctttaccttcagctacacttttgaggacgttcctttccacagcagctacgctcacagccagagtctggaccgtctcatgaatcctctcatcgaccagtacctgtattacttgagcagaacaaacactccaagtggaaccaccacgcagtcaaggcttcagttttctcaggccggagcgagtgacattcgggaccagtctaggaactggcttcctggaccctgttaccgccagcagcgagtatcaaagacacctgcggataacaacaacagtgaatactcgtggactggagctaccaagtaccacctcaatggcagagactctctggtgaatccgggcccggccatggcaagccacaaggacgatgaagaaaagttttttcctcagagcggggttctcatctttgggaagcaaggctcagagaaaacaaatgtggacattgaaaaggtcatgattacagacgaagaggaaatcaggacaaccaatcccgtggctacggagcagtatggttctgtatctaccaacctccagagaggcaacctagcaaaccaagactacacaaaaactgctaggcaagcagctaccgcagatgtcaacacacaaggcgttcttccaggcatggtctggcaggacagagatgtgtaccttcaggggcccatctgggcaaagattccacacacggacggacattttcacccctctcccctcatgggtggattcggacttaaacaccctcctccccagattctcatcaagaacaccccggtacctgcgaatccttcgaccaccttcagtgcggcaaagtttgcttccttcatcacacagtactccacgggacaggtcagcgtggagatcgagtgggagctgcagaaggaaaacagcaaacgctggaatcccgaaattcagtacacttccaactacaacaagtctattaatgtggactttactgtggacactaatggcgtgtattcagagcctcgccccattggcaccagatacctgactcgtaatctgtaa

SEQ ID NO: 78 - protein, 745 aa, synthetic construct
  REGION 1..745: note = synthetically generated sequence
MAADGYLPDWLEDTLSEGIRQWWKLKPGPPPPKPAERHKDDSRGLVLPGYKYLGPFNGLDKGEPVNAADAAALEHDKAYDRQLDSGDNPYLKYNHADAEFQERLKEDTSFGGNLGRAVFQAKKRVLEPLGLVEEPVKTAPGKKRPVEHSPVEPDSSSGTGKAGQQPARKRLNFGQTGDADSVPDPQPLGQPPAAPSGLGTNTMATGGGAPMADNNEGADGVGNSSGNWHCDSTWMGDRVITTSTRTWALPTYNNHLYKQISSQSGASNDNHYFGYSTPWGYFDFNRFHCHFSPRDWQRLINNNWGFRPKRLNFKLFNIQVKEVTQNDGTTTIANNLTSTVQVFTDSEYQLPYVLGSAHQGCLPPFPADVFMVPQYGYLTLNNGSQAVGRSSFYCLEYFPSQMLRTGNSFTFSYTFEDVPFHSSYAHSQSLDRLMNPLIDQYLYYLSRTNTPSGTTTQSRLQFSQAGASDIRDQSRNWLPGPCYRQQRVSKTPADNNNSEYSWTGATKYHLNGRDSLVNPGPAMASHKDDEEKFFPQSGVLIFGKQGSEKTNVDIEKVMITDEEEIRTTNPVATEQYGSVSTNLQRGNLANQDYTKTARQAATADVNTQGVLPGMVWQDRDVYLQGPIWAKIPHTDGHFHPSPLMGGFGLKHPPPQILIKNTPVPANPSTTFSAAKFASFITQYSTGQVSVEIEWELQKENSKRWNPEIQYTSNYNKSINVDFTVDTNGVYSEPRPIGTRYLTRNL

SEQ ID NO: 79 - DNA, 27 bp, synthetic construct
  misc_feature 1..27: note = synthetically generated sequence
  source 1..27: mol_type = other DNA
acgcggaagcttcgatcaactacgcag

SEQ ID NO: 80 - DNA, 32 bp, synthetic construct
  misc_feature 1..32: note = synthetically generated sequence
  source 1..32: mol_type = other DNA
agaccaaagttcaactgaaacgaattaaacgg

SEQ ID NO: 81 - protein, 10 aa, synthetic construct
  REGION 1..10: note = synthetically generated sequence
LAISDQTKHA

SEQ ID NO: 82 - protein, 10 aa, synthetic construct
  REGION 1..10: note = synthetically generated sequence
LAKDQTKSTA

SEQ ID NO: 83 - protein, 10 aa, synthetic construct
  REGION 1..10: note = synthetically generated sequence
LANQDYTKTA

SEQ ID NO: 84 - protein, 10 aa, synthetic construct
  REGION 1..10: note = synthetically generated sequence
LAHDITKNIA

SEQ ID NO: 85 - protein, 10 aa, synthetic construct
  REGION 1..10: note = synthetically generated sequence
LADQDYTKTA

SEQ ID NO: 86 - protein, 10 aa, synthetic construct
  REGION 1..10: note = synthetically generated sequence
LAQPDATKNA

SEQ ID NO: 87 - DNA, 25 bp, synthetic construct
  misc_feature 1..25: note = synthetically generated sequence
  source 1..25: mol_type = other DNA
caccgcaagggcgaggaggtcatca

SEQ ID NO: 88 - DNA, 25 bp, synthetic construct
  misc_feature 1..25: note = synthetically generated sequence
  source 1..25: mol_type = other DNA
aaactgatgacctcctcgcccttgc

SEQ ID NO: 89 - DNA, 26 bp, synthetic construct
  misc_feature 1..26: note = synthetically generated sequence
  source 1..26: mol_type = other DNA
caccgtggagggctccatgaacggcc

SEQ ID NO: 90 - DNA, 26 bp, synthetic construct
  misc_feature 1..26: note = synthetically generated sequence
  source 1..26: mol_type = other DNA
aaacggccgttcatggagccctccac

SEQ ID NO: 91 - DNA, 26 bp, synthetic construct
  misc_feature 1..26: note = synthetically generated sequence
  source 1..26: mol_type = other DNA
caccgaggacggcggccactacctgg

SEQ ID NO: 92 - DNA, 26 bp, synthetic construct
  misc_feature 1..26: note = synthetically generated sequence
  source 1..26: mol_type = other DNA
aaacccaggtagtggccgccgtcctc

SEQ ID NO: 93 - DNA, 26 bp, synthetic construct
  misc_feature 1..26: note = synthetically generated sequence
  source 1..26: mol_type = other DNA
caccgacaacaacatggccgtcatca

SEQ ID NO: 94 - DNA, 26 bp, synthetic construct
  misc_feature 1..26: note = synthetically generated sequence
  source 1..26: mol_type = other DNA
aaactgatgacggccatgttgttgtc

SEQ ID NO: 95 - DNA, 27 bp, synthetic construct
  misc_feature 1..27: note = synthetically generated sequence
  source 1..27: mol_type = other DNA
caccgaaggacggcggccactacctgg

SEQ ID NO: 96 - DNA, 27 bp, synthetic construct
  misc_feature 1..27: note = synthetically generated sequence
  source 1..27: mol_type = other DNA
aaacccaggtagtggccgccgtccttc

SEQ ID NO: 97 - DNA, 26 bp, synthetic construct
  misc_feature 1..26: note = synthetically generated sequence
  source 1..26: mol_type = other DNA
caccgacaacaacatggccgtcatca

SEQ ID NO: 98 - DNA, 26 bp, synthetic construct
  misc_feature 1..26: note = synthetically generated sequence
  source 1..26: mol_type = other DNA
aaactgatgacggccatgttgttgtc

SEQ ID NO: 99 - DNA, 25 bp, synthetic construct
  misc_feature 1..25: note = synthetically generated sequence
  source 1..25: mol_type = other DNA
caccggtcaccttcagcttggcggt

SEQ ID NO: 100 - DNA, 25 bp, synthetic construct
  misc_feature 1..25: note = synthetically generated sequence
  source 1..25: mol_type = other DNA
aaacaccgccaagctgaaggtgacc

SEQ ID NO: 101 - DNA, 25 bp, synthetic construct
  misc_feature 1..25: note = synthetically generated sequence
  source 1..25: mol_type = other DNA
caccgccgtacatgaactgggggga

SEQ ID NO: 102 - DNA, 24 bp, synthetic construct
  misc_feature 1..24: note = synthetically generated sequence
  source 1..24: mol_type = other DNA
aaactccccccagttcatgtacgg

SEQ ID NO: 103 - DNA, 26 bp, synthetic construct
  misc_feature 1..26: note = synthetically generated sequence
  source 1..26: mol_type = other DNA
caccgtcttgtaatcggggatgtcgg

SEQ ID NO: 104 - DNA, 26 bp, synthetic construct
  misc_feature 1..26: note = synthetically generated sequence
  source 1..26: mol_type = other DNA
aaacccgacatccccgattacaagac

SEQ ID NO: 105 - DNA, 25 bp, synthetic construct
  misc_feature 1..25: note = synthetically generated sequence
  source 1..25: mol_type = other DNA
caccgccgtcctgcagggaggagtc

SEQ ID NO: 106 - DNA, 25 bp, synthetic construct
  misc_feature 1..25: note = synthetically generated sequence
  source 1..25: mol_type = other DNA
aaacgactcctccctgcaggacggc

SEQ ID NO: 107 - protein, 10 aa, synthetic construct
  REGION 1..10: note = synthetically generated sequence
  REGION 3..4: note = misc_feature - Xaa can be any naturally occurring amino acid
  SITE 6: note = misc_feature - Xaa can be any naturally occurring amino acid
  SITE 9: note = misc_feature - Xaa can be any naturally occurring amino acid
LAXXDXTKXA

SEQ ID NO: 108 - protein, 10 aa, synthetic construct
  REGION 1..10: note = synthetically generated sequence
  SITE 3: note = misc_feature - Xaa can be any naturally occurring amino acid
  SITE 5: note = misc_feature - Xaa can be any naturally occurring amino acid
  REGION 8..9: note = misc_feature - Xaa can be any naturally occurring amino acid
LAXDXTKXXA